European Patent Specification EP 3 624 896 B1, published July 15, 2026. Title: COMPOSITIONS AND METHODS FOR TREATING CANCER WITH ATYPICAL BRAF MUTATIONS. Applicant: Biomed Valley Discoveries, Inc. Application US 62/506,995. The sequence listing filed with the application follows.

SEQUENCE LISTING (44 sequences)

SEQ ID NO: 1 - DNA, 2949 bp, Homo sapiens
cgcctcccttccccctccccgcccgacagcggccgctcgggccccggctctcggttataagatggcggcgctgagcggtggcggtggtggcggcgcggagccgggccaggctctgttcaacggggacatggagcccgaggccggcgccggcgccggcgccgcggcctcttcggctgcggaccctgccattccggaggaggtgtggaatatcaaacaaatgattaagttgacacaggaacatatagaggccctattggacaaatttggtggggagcataatccaccatcaatatatctggaggcctatgaagaatacaccagcaagctagatgcactccaacaaagagaacaacagttattggaatctctggggaacggaactgatttttctgtttctagctctgcatcaatggataccgttacatcttcttcctcttctagcctttcagtgctaccttcatctctttcagtttttcaaaatcccacagatgtggcacggagcaaccccaagtcaccacaaaaacctatcgttagagtcttcctgcccaacaaacagaggacagtggtacctgcaaggtgtggagttacagtccgagacagtctaaagaaagcactgatgatgagaggtctaatcccagagtgctgtgctgtttacagaattcaggatggagagaagaaaccaattggttgggacactgatatttcctggcttactggagaagaattgcatgtggaagtgttggagaatgttccacttacaacacacaactttgtacgaaaaacgtttttcaccttagcattttgtgacttttgtcgaaagctgcttttccagggtttccgctgtcaaacatgtggttataaatttcaccagcgttgtagtacagaagttccactgatgtgtgttaattatgaccaacttgatttgctgtttgtctccaagttctttgaacaccacccaataccacaggaagaggcgtccttagcagagactgccctaacatctggatcatccccttccgcacccgcctcggactctattgggccccaaattctcaccagtccgtctccttcaaaatccattccaattccacagcccttccgaccagcagatgaagatcatcgaaatcaatttgggcaacgagaccgatcctcatcagctcccaatgtgcatataaacacaatagaacctgtcaatattgatgacttgattagagaccaaggatttcgtggtgatggaggatcaaccacaggtttgtctgctaccccccctgcctcattacctggctcactaactaacgtgaaagccttacagaaatctccaggacctcagcgagaaaggaagtcatcttcatcctcagaagacaggaatcgaatgaaaacacttggtagacgggactcgagtgatgattgggagattcctgatgggcagattacagtgggacaaagaattggatctggatcatttggaacagtctacaagggaaagtggcatggtgatgtggcagtgaaaatgttgaatgtgacagcacctacacctcagcagttacaagccttcaaaaatgaagtaggagtactcaggaaaacacgacatgtgaatatcctactcttcatgggctattccacaaagccacaactggctattgttacccagtggtgtgagggctccagcttgtatcaccatctccatatcattgagaccaaatttgagatgatcaaacttatagatattgcacgacagactgcacagggcatggattacttacacgccaagtcaatcatccacagagacctcaagagtaataatatatttcttcatgaagacctcacagtaaaaataggtgattttggtctagctacagtgaaatctcgatggagtgggtcccatcagtttgaacagttgtctggatccattttgtggatggcaccagaagtcatcagaatgcaagataaaaatccatacagctttcagtcagatgtatatgcatttggaattgttctgtatgaattgatgactggacagttaccttattcaaacatcaacaacagggaccagataatttttatggtgggacgaggatacctgtctccagatctcagtaaggtacggagtaactgtccaaaagccatgaagagattaatggcagagtgcctcaaaaagaaaagagatgagagaccactctttccccaaattctcgcctctattgagctgctggcccgctcattgccaaaaattcaccgcagtgcatcagaaccctccttgaatcgggctggtttccaaacagaggattttagtctatatgcttgtgcttctccaaaaacacccatccaggcagggggatatggtgcgtttcctgtccactgaaacaaatgagtgagagagttcaggagagtagcaacaaaaggaaaataaatgaacatatgtttgcttatatgttaaattgaataaaatactctctttttttttaaggtgaaccaaagaacacttgtgtggttaaagactagatataatttttccccaaactaaaatttatacttaacattggatttttaacatccaagggttaaaatacatagacattgctaaaaattggcagagcctcttctagaggctttactttctgttccgggtttgtatcattcacttggttattttaagtagtaaacttcagtttctcatgcaacttttgttgccagctatcacatgtccactagggactccagaagaagaccctacctatgcctgtgtttgcaggtgagaagttggcagtcggttagcctgggttagataaggcaaactgaacagatctaatttaggaagtcagtagaatttaataattctattattattcttaataatttttctataactatttctttttataacaatttggaaaatgtggatgtcttttatttccttgaagcaataaactaagtttctttttataaaaa

SEQ ID NO: 2 - protein, 766 aa, Homo sapiens [sequence omitted]

SEQ ID NO: 3 - DNA, 3906 bp, Rattus norvegicus
atggcggcgctgagtggcggcggtggcagcagcagcggtggcggtggcggcggcggcggcggcggtggtggcggcggcggcggcggcgccgaacagggacaggctctgttcaatggcgacatggagccggaggccggcgctggcgccgcggcctcttcggccgcggacccggccattcctgaagaggtgtggaatatcaagcaaatgattaagttgacacaggaacatatagaggccctattggacaagtttggtggggagcataacccaccgtcaatatacctggaggcctatgaagagtacaccagcaagctagatgcccttcagcagagagagcagcagctgttggaatccctggtttttcaaactcccacagatgtatcacggaacaaccccaagtcaccacagaaacctatcgttcgtgtcttcctgcccaacaaacagaggacagtggtgcccgcaagatgtggtgtaacggtccgagacagtctaaagaaagcactaatgatgaggggtctcatcccagagtgctgtgctgtttacagaattcaggacggagagaagaaaccaattggctgggacactgacatttcctggcttactggagaggagctacatgttgaagtactagagaatgttcctctgacaacccacaacttcgtacggaaaacttttttcaccttagcattttgtgacttttgccgaaagctgcttttccagggtttccgctgtcaaacatgtggttataagtttcaccagcgttgtagtacagaggttccactgatgtgtgttaattatgaccaacttgatttgctgtttgtctccaagttctttgagcatcacccagtaccacaggaggaggccttctcagcagagactacccttccatctggatgctcttccgcacccccctcagactctattgggccccaaatcctcaccagtccatctccttcaaaatccattccaattccacagcccttccggccagcagatgaagatcatcgcaatcagtttgggcaacgagaccgctcctcctccgctcccaatgttcatataaacacaatcgaacctgtcaatattgatgaaaaattcccagaagtggaattacaggatcaaagggatttgattagagaccaggggtttcgtggggatggagcccctttgaaccagctgatgcgctgtcttcggaaataccaatcccggactcccagccccctcctccattctgtccccagtgaaatagtgtttgattttgagcctggcccagtgttcagagggtcaaccacaggcttgtcggccaccccacctgcctcattacctggctcactcactaacgtgaaagccttacagaaatctccaggacctcagcgggaaaggaagtcctcctcctcctcctcctccacggaagacagaagtcggatgaaaacacttggtagaagagattcaagtgatgattgggagattcctgatggacagattacagtgggacagagaattggatctgggtcctttggaactgtctacaagggaaagtggcatggcgacgtggcagtgaaaatgctgaatgtgacagcacccacacctcagcagttacaggccttcaaaaacgaagtcggagtactcaggaaaactcgacatgtgaacatcctccttttcatgggctattctacaaagccacagctggctattgttacacagtggtgtgaaggctccagcttatatcaccatctccacatcattgagaccaaatttgagatgatcaaacttatagatattgcacggcagactgcacagggcatggattacttacacgccaagtcaatcatccacagagacctcaagagtaataatatatttcttcatgaagacctcacggtaaaaataggtgactttggtttagccacagtgaagtcccgatggagtgggtcccatcagtttgaacagttgtctggatctattttgtggatggcacccgaagtaatcagaatgcaagataaaaacccatatagctttcagtcagacgtgtatgcatttgggattgttctgtatgaactgatgactggtcagctaccttattcaaacatcaacaacagggatcagataatttttatggtgggacgaggatacctatctccagatctcagtaaggtacggagtaactgtccaaaagccatgaagagattaatggcagagtgcctcaaaaagaaaagagacgagagaccactctttccccaaattctcgcctctattgagctgctggcccgctcattgccaaaaattcaccgcagtgcatcagaaccctccttgaatcgggctggtttccaaacagaagattttagtctgtatgcttgtgcttctccaaaaacacccatccaagcagggggatatggagaatttgcagccttcaagtagccactccatcatggcagcatctactctttatttcttaagtcttgtgttcatacaatttgttaacatcaaaacacagttctgttcctcaaattttttttaaagatacaaaattttcaatgcataagctcgtgtggaacagaatggaatttcctattcaacaaaagagggaagaatgttttaggaaccagaattctctgctgcccgtgtttcttcttcaacacaaatatcatgtgcatacaactctgcccattcccaagaagaaagaggagagaccccgaattctgcccttttggtggtcaggcatgatggaaagaatttgctgctgcagcttgggaaaaattgctatggaaagtctgccagtcaactttgcccttctaaccaccagatccatttgtggctggtcatctgatggggcgatttcaatcaccaagcatcgttcttgcctgttgtgggattatgtcgtggagcactttccctatccaccaccgttaatttccgagggatggagtaaatgcagcataccctttgtgtagcacctgtccagtcctcaaccaatgctatcacagtgaagctctttaaatttaagtggtgggtgagtgttgaggagagactgccttgggggcagagaaaaggggatgctgcatcttcttcctcacctccagctctctcacctcgggttgccttgcacactgggctccgcctaaccactcgggctgggcagtgctggcacacattgccgccttttctcattgggtccagcaattgagcagagggttgggggattgtttcctccacaatgtagcaaattctcaggaaaatacagtccatatcttcctctcagctcttccagtcaccaaatacttacgtggctcctttgtccaggacataaaacaccgtggacaacacctaattaaaagcctacaaaactgcttactgacagttttgaatgtgagacatttgtgtaatttaaatgtaaggtacaggtcttaatttcttctattaagtttcttctatttttatttaaacgaagaaaataattttcaggtttaattggaataaacgaatacttcccaaaagactatataccctgaaaattatatttttgttaattgtaaacaacttttaaaaaatggttattatccttttctctacctaaaattatgggaaatcttagcataatgacaattatttatactttttaaataaatggtacttgctggatccacactaacatctttgctaacattcccattgtttcttccaacttcactcctacactacatcctccatcctctttctagtcttttatctataatatgcaacctaaaataaaagtggtggtgtctccattcattcttcttcttccttttttccccaagcctggtcttcaaaaggttgggtaatttagtagctgagttccctaggtagaaatagaactattagggacattggggttgtaggaaagcgtgaggcctgtcaccagttgttctt

SEQ ID NO: 4 - protein, 804 aa, Rattus norvegicus
MAALSGGGGSSSGGGGGGGGGGGGGGGGGAEQGQALFNGDMEPEAGAGAAASSAADPAIPEEVWNIKQMIKLTQEHIEALLDKFGGEHNPPSIYLEAYEEYTSKLDALQQREQQLLESLVFQTPTDVSRNNPKSPQKPIVRVFLPNKQRTVVPARCGVTVRDSLKKALMMRGLIPECCAVYRIQDGEKKPIGWDTDISWLTGEELHVEVLENVPLTTHNFVRKTFFTLAFCDFCRKLLFQGFRCQTCGYKFHQRCSTEVPLMCVNYDQLDLLFVSKFFEHHPVPQEEAFSAETTLPSGCSSAPPSDSIGPQILTSPSPSKSIPIPQPFRPADEDHRNQFGQRDRSSSAPNVHINTIEPVNIDEKFPEVELQDQRDLIRDQGFRGDGAPLNQLMRCLRKYQSRTPSPLLHSVPSEIVFDFEPGPVFRGSTTGLSATPPASLPGSLTNVKALQKSPGPQRERKSSSSSSSTEDRSRMKTLGRRDSSDDWEIPDGQITVGQRIGSGSFGTVYKGKWHGDVAVKMLNVTAPTPQQLQAFKNEVGVLRKTRHVNILLFMGYSTKPQLAIVTQWCEGSSLYHHLHIIETKFEMIKLIDIARQTAQGMDYLHAKSIIHRDLKSNNIFLHEDLTVKIGDFGLATVKSRWSGSHQFEQLSGSILWMAPEVIRMQDKNPYSFQSDVYAFGIVLYELMTGQLPYSNINNRDQIIFMVGRGYLSPDLSKVRSNCPKAMKRLMAECLKKKRDERPLFPQILASIELLARSLPKIHRSASEPSLNRAGFQTEDFSLYACASPKTPIQAGGYGEFAAFK

SEQ ID NO: 5 - DNA, 9728 bp, Mus musculus
ccctcaggctcggctgcgccggggccgccggcgggttccagaggtggcctccgccccggccgctccgcccacgccccccgcgcctccgcgcccgcctccgcccgccctgcgcctcccttccccctccccgccccgcggcggccgctcggcccggctcgcgcttcgaagatggcggcgctgagtggcggcggtggcagcagcagcggtggcggcggcggcggtggcggcggcggtggcggtggcgacggcggcggcggcgccgagcagggccaggctctgttcaatggcgacatggagccggaggccggcgctggcgccgcggcctcttcggctgcggacccggccattcctgaagaggtatggaatatcaagcaaatgattaagttgacacaggaacatatagaggccctattggacaaatttggtggagagcataacccaccatcaatatacctggaggcctatgaagagtacaccagcaagctagatgcccttcagcaaagagaacagcagcttttggaatccctggtttttcaaactcccacagatgcatcacggaacaaccccaagtcaccacagaaacctatcgttagagtcttcctgcccaacaaacagaggacagtggtacccgcaagatgtggtgttacagttcgagacagtctaaagaaagcactgatgatgagaggtctcatcccagaatgctgtgctgtttacagaattcaggatggagagaagaaaccaattggctgggacacggacatttcctggcttactggagaggagttacatgttgaagtactggagaatgtcccacttacaacacacaactttgtacggaaaacttttttcaccttagcattttgtgacttttgccgaaagctgcttttccagggtttccgttgtcaaacatgtggttataaatttcaccagcgttgtagtacagaggttccactgatgtgtgtaaattatgaccaacttgatttgctgtttgtctccaagttctttgagcatcacccagtaccacaggaggaggcctccttcccagagactgcccttccatctggatcctcttccgcacccccctcagactctactgggccccaaatcctcaccagtccatctccttcaaaatccattccaattccacagcccttccgaccagcagatgaagatcatcgcaatcagtttgggcaacgagaccggtcctcctcagctcccaatgttcatataaacacaattgagcctgtgaatatcgatgaaaaattcccagaagtggaattacaggatcaaagggatttgattagagaccaggggtttcgtggtgatggagcccccttgaaccaactgatgcgctgtcttcggaaataccaatcccggactcccagccccctcctccattctgtccccagtgaaatagtgtttgattttgagcctggcccagtgttcagagggtcaaccacaggcttgtccgccaccccgcctgcctcattacctggctcactcactaacgtgaaagccttacagaaatctccaggtcctcagcgggaaaggaagtcatcttcttcctcatcctcggaggacagaagtcggatgaaaacacttggtagaagagattcaagtgatgactgggagattcctgatggacagattacagtgggacagagaattggatctgggtcatttggaactgtctacaagggaaagtggcatggtgatgtggcagtgaaaatgttgaatgtgacagcacccacacctcaacagctacaggccttcaaaaatgaagtaggagtgctcaggaaaactcgacatgtgaatatcctccttttcatgggctattctacaaagccacaactggcaattgttacacagtggtgtgagggctccagcttatatcaccatctccacatcattgagaccaaatttgagatgatcaaacttatagatattgctcggcagactgcacagggcatggattacttacacgccaagtcaatcatccacagagacctcaagagtaataatatatttcttcatgaagacctcacggtaaaaataggtgactttggtctagccacagtgaaatctcggtggagtgggtcccatcagtttgaacagttgtctggatctattttgtggatggcaccagaagtaatcagaatgcaagataaaaacccgtatagctttcagtcagacgtgtatgcgtttgggattgttctgtacgaactgatgaccggccagctaccttattcaaacatcaacaacagggatcagataatttttatggtgggacgaggatacctatctccagatctcagtaaggtacggagtaactgtccaaaagccatgaagagattaatggcagagtgcctcaaaaagaaaagagacgagagaccactctttccccaaattctcgcctccattgagctgctggcccgctcattgccaaaaattcaccgcagtgcatcagaaccttccttgaatcgggctggtttccaaacagaagattttagtctgtatgcttgtgcttctccgaaaacacccatccaagcagggggatatggagaatttgcagccttcaagtagccagtccatcatggcagcatctactctttatttcttaagtcttgtgttcatacagtttgttaacatcaaaacacagttctgttcctcaaaaaattttttaaagatacaaaattttcaatgcataagttcatgtggaacagaatggaatttcctattcaacaaaagagggaagaatgttttaggaaccagaattctctgctgcccgtgtttcttcttcaacataactatcacgtgcatacaagtctgcccattcccaagaagaaagaggagagaccctgaattctgcccttttggtggtcaggcatgatggaaagaatttgctgctgcagcttgggaaaattgctatggaaagtctgccagtcgactttgcccttctaaccaccagatcagcctgtggctggtcatctgatggggcgatttccatcaccaagcatcgttcttgcctattctgggattatgttgtggagcactttccctgtccagcaccgttcatttctgagggatggagtaaatgcagcattcccttgtgtagcgcctgttcagtcctcagcagctgctgtcacagcgaagctttttacagttaagtggtgggggagagttgaggagagcctgcctcggggcagagaaaagggggtgctgcatcttcttcctcacctccagctctctcacctcgggttgccttgctcactgggctccgcctaaccactcaggctgctcagtgctggcacacattgccttcttttctcattgggtccagcaattgaggagagggttgggggattgtttcctcctcaatgtagcaaattctcaggaaaatacagtccatatcttcctctcagctcttccagtcaccaaatacttacgtggctcctttgtccaggacataaaacaccgtggacaacacctaattaaaagcctacaaaactgcttactgacagttttgaatgtgagacacttgtgtaatttaaatgtaaggtacaggttttaatttctgagtttcttctatttttatttaaaagaagaaaataattttcagttttaattggaataaatgagtacttcccacaagactatataccctgaaaattatatttttgttaattgtaaacaacttttaaagaataattattatccttttctctacctaaaaattatggggaatcttagcataatgacaattatttatactttttaaataaatggtacttgctggatccacactaacatctttgctaacaatcccattgtttcttccaacttaactcctacactacatcctacatcctctttctagtcttttatctataatatgcaacctaaaataaacgtggtggcgtctccattcattctccctcttcctgttttccccaagcctggtcttcaaaaggttgggtaatcggtccctgagctccctagctggcaatgcaactattagggacattggagttgcaggagagcaggaagcctgtccccagctgttcttctagaaccctaaatcttatctttgcacagatcaaaagtatcacctcgtcacagttctccttagcctttacttacaggtaatataaataaaaatcaccatagtagtaaagaaaacaactggatggattgatgaccagtacctctcagagccaggaatcttgaatctccaggatttatacgtgcaaatttaaggagatgtacttagcaacttcaagccaagaacttccaaaatactagcgaatctaaaataaaatggaattttgagttatttttaaagttcaaattataattgataccactatgtatttaagcctactcacagcaagttagatggattttgctaaactcattgccagactgtggtggtggtggtggtagtgtgcacctttaatccaagcaactcagcaatcagaatgaggtaaatctctgtgaatacaaggcctgcctagtctgcagcgctagttccaggatagccagggctacacacacaaaaaccctctctcaaaaaaaacaaaattaattagttgataataaaaaataactaaagtatcatcaaaggaaggcctactggaagttttatatattcccagtaaattgaaaaatattctgaagttattaaccagttagcaacaatgtgtttttaagtcttacataaacagagcaaagtcttcaaatgtttcagagctgagaagataattgtgcttgatatgaaaaatagcctctccatatgatgtgccacattgaaaggcgtcattacccttttaaatacttcttaatgtggctttgttccctttacccaggattagctagaaagagctaggtaggcttcggccacagttgcacatttcgggcctgctgaagaatgggagctttgaaggctggccttggtggaggagcccctcagtgctggagggtggggcgtgtacgcagcatggaagtggtctagacagagtgcaaagggacagacttctttctcattttagtatagggtgatgtctcacttgaaatgagaaagtagagttgatattaaacgaagctgtgcccagaaaccaggctcagggtattgtgagattttctttttaaatagagaatataaaagatagaaataaatatttaaaccttccttcttattttctatcaaatagattttttttatcatttgcaaacaacataaaaaaaggtttcttttgtggggttttctttccttcttttttttttttttttttttttaagactgcagataatcttgttgagctcctcggaaaatacaaggaagtccgtgtttgtgcagagcgctttatgagtaactgtatagacagtgtggctgcttcactcatcccagagggctgcagctgtcggcccatgaagtggctgcagtgcctcgtgagatctgctttgttttgtttggagtgaagtctttgaaaggtttgagtgcaactatataggactgtttttaaataagtagtattcctcatgaactttctcattgttaagctacaggacccaaactctaccactaagatattattaacctcaaaatgtagtttatagaaggaatttgcaaatagaatatccagttcgtacttatatgcatcttcaacaaagattctctgtgacttgttggatttggttcctgaacagcccatttctgtatttgaggttaggagggcataatgaggcatcctaaaagacaatctgatataaactgtatgctagatgtatgctggtaggggagaaagcattctgtaaagacatgatttaagacttcagctctgtcaaccagaaaccttgtaaatacttcctgtcttggtgcagccccgcccctttgatcacacgatgttgtcttgtgcttgtcagacactgtcagagctgctgttcgtccctctgcagatctcacctgtccccactgcacacccacctcctgcctcttgcagacctcagcatctagctttagttggaaacagttcagggttcaggtgacttcttaaaaaaaaaaaaaaaccctacctcctcagaatgaggtaatgaatagttatttatttaaagtatgaagagtcaggagcgctcgaacatgaaggtgatttaagatggttcctttcgtgtgtattgtagctgagcacttgtttttgtcctaaagggcattatacatttaagcagtgattctgtttaaagatgtttttctttaaaggtgtagctcagagtatctgttgttggaattggtgccagagtctgcttaatagatttcagaatcctaagcttaagtcagtcgcatgaagttaagtagttatggtaacactttgctagccatgatataattctactttttaggagtaggtttggcaaaactgtatgccttcaaagtgagttggccacagctttgtcacatgcacagatactcatctgaagagactgcccagctaagagggcggaaggatacccttttttcctacgattcgcttctttgtccacgttggcattgttagtactagtttatcagcaccttgaccagcagatgtcaaccaataagctatttttaaaaccatagccagagatggagaggtcactgtgagtagaaacagcaggacgcttacaggagtgaaatggtgtagggaggctctagaaaaatatcttgacaatttgccaaatgatcttactgtgccttcatgatgcaataaaaaagctaacattttagcagaaatcagtgatttacgaagagagtggccagtctggtttaactcagctgggataatatttttagagtgcaatttagactgcgaagataaatgcactaaagagtttatagccaattcacatttgaaaaataagaaaatggtaaattttcagtgaaatatttttttaaagcacataatccctagtgtagccagaaatatttaccacatagagcagctaggctgagatacagtccagtgacatttctagagaaaccttttctactcccacgggctcctcaaagcatggaaattttatacaaaatgtttgacattttaagatactgctgtagtttagttttgaaatagtatgtgctgagcagcaatcatgtactaactcagagagagaaaacaacaacaaattgtgcatctgatttgttttcagagaaatgctgccaacttagatactgagttctcagagcttcaagtgtaaacttgcctcccaagtcctgtttgcaaatgaagttggctagtgctactgactgctccagcacatgatggaaggcagggggctgtctctgaagtgtcttctataaagggacaatagaatagtgagagacctggtcagtgtgtgtcagctggacactccatgctatgggacttgcatcttctgtcctcaccatccccaagacattgtgctttcctcagttgtcctctagctgtttcactcagacaccaagatgaattactgatgccagaaggggccaaaatggccagtgtgttttgggggttgtatcagttgactggacaataactttaatagtttcagatcatttatttttacttccattttgacagacatttaaatggaaatttagtcctaacttttgtcatttgaaaggaaaaattaacagttcctataagatacttttgaggtggaatctgacatcctaattttttttcttttcagtgggtttgcagcgagggtcttgtatgcactaggcaagggttctaccactaagccacatttcccaggaaataaaatgttaacagttaaaacatacacacaaatacacaaacaccttattaccactttagtaaagtgagagatgtgcgtcctttgtctcagtctccacgatttcagctgccccttgtatgaataactcagtctcgctaaactgtttacttttatttacctggtttgactagttgcagctatataaccagttgtgcatgaggacaacagccagtgtgtttgttttgtttttggttttttgtggtacattttttgtaaagaattctgtagattgaagtgctctttgaaaacagaactgagatatatttattcttgttagcatcaaaaaacattttgtgcaaatgatttgcttttcctggcaggctgagtaccatatccagcgcccacaattgcgggttcccatctaccatgtccacaggggagacagacgggaagcacatgaggggtgtgtttacagagttgtaggagttatgtagttctcttgttgccttggaaatcactgttgttttaagactgttgaacccgtgtgtttggctgggctgtgagttacatgaagaaactgcaaactagcatatgcagacaaagctcacagactaggcgtaaatggaggaaaatggaccaaaataaggcagggtgacacataaaccttgggcttcggagaaaactaagggtggagatgaactataatcacctgaatacaatgtaagagtgcaataagtgtgcttattctaagctgtgaacttcttttaaatcattcctttctaatacatttatgtatgttccattgctgactaaaaccagctatgagaacatatgcctttttattcatgttaactaccagtttaagtggctaaccttaatgtcttatttatcttcattttgtattagtttacataccaggtatgtgtgtgtgctgtactcttcttccctttatttgaaaacacttttcactgggtcatctccttggccattccacaacacaactttggtttggctttcaatgtcaccttatttgatggcctgtgtcccagtagcagaatttatggtattcccattgctggctgctcttccgaccctttgcttctacagcacttgtctctcctaagatagtcagaaactaactgatcaggggatggacttcaccattcatcgtgtctcttcaattctattaaatagaccactcttgggctttagaccaggaaaaaggagacagctctagccatctaccaagcctcaccctaaaaggtcacccgtacttcttggtctgaggacaagtctccactccagtaagggagaggggaggaaatgcttcctgtttgaaatgcagtgaattcctatggctcctgtttcaccacccgcacctatggcaacccatatacattcctcttgtctgtaactgccaaaggttgggtttatgtcacttcagttccactcaagcattgaaaaggttctcatggagtctggggtgtgcccagtgaaaagatggggactttttcattatccacagacctctctatacctgctttgcaaaaattataatggagtaactatttttaaagcttatttttcaattcataagaaaaagacatttattttcaatcaaatggatgatgtctcttatcccttatccctcaatgtttgcttgaattttgtttgttccctatacctactccctaattctttagttccttcctgctcaggtcccttcatttgtactttggagtttttctcatgtaaatttgtataatggaaaatattgttcagtttggatagaaagcatggagaaataaataaaaaaagatagctgaaaatcaaattgaagaaatttatttctgtgtaaagttatttaaaaactctgtattatatttaaagaaaaaagcccaaccccccaaaaagtgctatgtaattgatgtgaatatgcgaatactgctataataaagattgactgcatggagaaa

SEQ ID NO: 6 - protein, 804 aa, Mus musculus
MAALSGGGGSSSGGGGGGGGGGGGGDGGGGAEQGQALFNGDMEPEAGAGAAASSAADPAIPEEVWNIKQMIKLTQEHIEALLDKFGGEHNPPSIYLEAYEEYTSKLDALQQREQQLLESLVFQTPTDASRNNPKSPQKPIVRVFLPNKQRTVVPARCGVTVRDSLKKALMMRGLIPECCAVYRIQDGEKKPIGWDTDISWLTGEELHVEVLENVPLTTHNFVRKTFFTLAFCDFCRKLLFQGFRCQTCGYKFHQRCSTEVPLMCVNYDQLDLLFVSKFFEHHPVPQEEASFPETALPSGSSSAPPSDSTGPQILTSPSPSKSIPIPQPFRPADEDHRNQFGQRDRSSSAPNVHINTIEPVNIDEKFPEVELQDQRDLIRDQGFRGDGAPLNQLMRCLRKYQSRTPSPLLHSVPSEIVFDFEPGPVFRGSTTGLSATPPASLPGSLTNVKALQKSPGPQRERKSSSSSSSEDRSRMKTLGRRDSSDDWEIPDGQITVGQRIGSGSFGTVYKGKWHGDVAVKMLNVTAPTPQQLQAFKNEVGVLRKTRHVNILLFMGYSTKPQLAIVTQWCEGSSLYHHLHIIETKFEMIKLIDIARQTAQGMDYLHAKSIIHRDLKSNNIFLHEDLTVKIGDFGLATVKSRWSGSHQFEQLSGSILWMAPEVIRMQDKNPYSFQSDVYAFGIVLYELMTGQLPYSNINNRDQIIFMVGRGYLSPDLSKVRSNCPKAMKRLMAECLKKKRDERPLFPQILASIELLARSLPKIHRSASEPSLNRAGFQTEDFSLYACASPKTPIQAGGYGEFAAFK

SEQ ID NO: 7 - DNA, 2232 bp, Oryctolagus cuniculus
atggggaatgtgtggaatatcaaacaaatgattaagttgacacaggagcatatagaggccctattggacaaatttggtggggagcataatccaccatcaatatatctggaggcctacgaagaatacaccagcaagctagatgccctccaacaaagagaacagcagttattggaatccctagtttttcaaaatcccacagatgtgtcacggagcaaccccaagtcaccacaaaaacctattgttagagtcttcctgcccaacaaacagaggacagtggtacctgcaagatgtggagttacggttcgagacagtctaaagaaagcgctgatgatgagaggtctgatcccagaatgctgtgctgtttacagaattcaggatggagagaagaagccaattggctgggacactgatatttcctggctcactggagaagagctgcatgtggaagtgttagagaatgtcccactcaccacacataactttgtacggaaaacttttttcaccttagcattttgtgacttctgtagaaagctgcttttccagggtttccgctgtcaaacatgtggctacaaatttcaccagcgttgtagtacggaagttccactgatgtgtgttaattatgaccaacttgatttgctgtttgtctccaagttctttgaacaccacccagtaccacaggaggaggcctccttagcagagactgccctcacatctgggtcatcgccttccgcacctccctcagactctattgggcaccaaattctcaccagtccgtccccttcaaaatccattccgattccacagtccttccgaccagcagatgaagatcatcgaaatcagtttgggcaacgagaccggtcttcatcagcgcctaatgttcacattaacacaatagaacctgtcaatattgatgaaaaattcccagaagtggaattacaggatcaaagggacttgattagagaccaagggtttcgtggtgatggagcccctttgaaccagctgatgcgctgtcttcggaaataccaatcccggactcccagtcccctcctaccttctgtccccagtgacatagtgtttgattttgagcctggcccagtgttcagaggatcgaccacgggtttgtctgccactccccctgcctcattacctggctcactcactagtgtgaaagctgtacagagatccccaggacctcagcgagagaggaagtcgtcttcctcctcagaagacaggaatcgaatgaaaactcttggtagacgggattcaagtgatgattgggagattcctgatgggcagatcaccgtgggacagagaattggatctggatcatttggaaccgtctacaagggaaaatggcacggtgatgtggcagtaaaaatgttgaatgtgacagcacctacacctcagcagttacaggccttcaaaaatgaagtaggagtactcaggaaaacacgacatgtgaatatcctacttttcatgggctattccacaaagccacagctggctattgttacccagtggtgtgagggctccagtttatatcaccatctccacatcattgagaccaaattcgagatgatcaaacttatagatattgcacggcagactgcacagggcatggattacttacacgccaagtcaatcatccacagagacctcaagagtaataatatatttcttcatgaagacctcacagtaaaaataggtgattttggtctagccacagtgaaatctcgatggagtgggtcccatcagtttgaacaattgtctggatccattttgtggatggcaccagaagtaatcagaatgcaagacaaaaacccatatagctttcagtcagatgtatatgcatttgggattgttctgtatgaattgatgactgggcagttaccttactcaaacatcaacaacagggaccagatcatttttatggtgggacgtggctacctgtctccagacctcagtaaggtacggagtaactgtccgaaagccatgaagagattaatggcagagtgcctcaaaaagaaaagagatgagagaccactctttccccaaattctcgcctccattgagctgctggcccgctcattgccaaaaatccaccgcagtgcatcagaaccctccttgaatcgggctggtttccagacagaggattttagtctatatgcttgtgcttctccaaaaacacccatccaggcagggggatatggagaatttgcagccttcaagtag

SEQ ID NO: 8 - protein, 743 aa, Oryctolagus cuniculus
MGNVWNIKQMIKLTQEHIEALLDKFGGEHNPPSIYLEAYEEYTSKLDALQQREQQLLESLVFQNPTDVSRSNPKSPQKPIVRVFLPNKQRTVVPARCGVTVRDSLKKALMMRGLIPECCAVYRIQDGEKKPIGWDTDISWLTGEELHVEVLENVPLTTHNFVRKTFFTLAFCDFCRKLLFQGFRCQTCGYKFHQRCSTEVPLMCVNYDQLDLLFVSKFFEHHPVPQEEASLAETALTSGSSPSAPPSDSIGHQILTSPSPSKSIPIPQSFRPADEDHRNQFGQRDRSSSAPNVHINTIEPVNIDEKFPEVELQDQRDLIRDQGFRGDGAPLNQLMRCLRKYQSRTPSPLLPSVPSDIVFDFEPGPVFRGSTTGLSATPPASLPGSLTSVKAVQRSPGPQRERKSSSSSEDRNRMKTLGRRDSSDDWEIPDGQITVGQRIGSGSFGTVYKGKWHGDVAVKMLNVTAPTPQQLQAFKNEVGVLRKTRHVNILLFMGYSTKPQLAIVTQWCEGSSLYHHLHIIETKFEMIKLIDIARQTAQGMDYLHAKSIIHRDLKSNNIFLHEDLTVKIGDFGLATVKSRWSGSHQFEQLSGSILWMAPEVIRMQDKNPYSFQSDVYAFGIVLYELMTGQLPYSNINNRDQIIFMVGRGYLSPDLSKVRSNCPKAMKRLMAECLKKKRDERPLFPQILASIELLARSLPKIHRSASEPSLNRAGFQTEDFSLYACASPKTPIQAGGYGEFAAFK

SEQ ID NO: 9 - DNA, 2186 bp, Cavia porcellus
atggcggcgctcagcggcggcggtggcgcggagcagggccaggctctgttcaacggggacatggagctcgaggccggcgccggcgccgcagcctcttcggctgcagaccctgccattcccgaggaggtatggaatatcaaacaaatgattaagttgacgcaggaacacatagaggccctattggacaaatttggtggagagcataatccaccatcaatatacctggaggcctatgaagaatacaccagcaaactagatgccctccaacaaagagaacagcagttactggaatccctcgggaatggaactgatttttctgtttctagctctgcatcactggacaccgttacatcttcttcttcttctagcctttcagtactaccttcatctctttcagtttttcaaaatcctacagatgtgtcacggagcaaccccaaatcaccacaaaaacctattgttagagtcttcctgcccaacaaacagaggacagtggtacctgcaaggtgtggagttacagtccgagacagtctgaagaaagcactcatgatgagaggtcttatcccagagtgctgtgctgtgtacagaattcaggatggagaaaagaaaccaattggctgggacactgacatttcctggcttactggggaagaattacatgtagaagtattggagaatgttccacttacaacacacaattttgtatgtatctttatattttttttgctgtttgtctccaagttctttgaacaccacccaataccacaggaggaggcttccttagcagagaccacccttacatctggatcatccccttctgcacccccctcagagtccattgggcccccaattctcaccagcccatctccttcaaaatccattccaattccacagcctttccggccaggagaggaagatcatcgaaatcaatttgggcagcgagaccggtcctcatctgctcccaatgtgcatataaacacaatagaacctgtcaatattgatgatttgattagagaccaagggtttcgtagtgatggaggatcaactacaggtttgtctgccaccccacctgcctcattacctggctcactcactaatgtgaaagccttacagaaatctccaggacctcagcgagaaaggaagtcatcttcatcctcagaagacagaaatcgaatgaaaacgcttggtagacgggactcaagtgatgattgggagattcctgatgggcagattacagtgggacaaagaattggatctgggtcatttggaacagtctacaaggggaagtggcatggtgacgtggcagtgaaaatgttgaatgtgacagcacccacacctcaacagttacaggccttcaaaaatgaagtaggagtactcaggaaaacacgacatgtgaatatcctactcttcatgggctattccacaaagccacagctagctattgttacccagtggtgtgagggctccagcttataccaccatctccacatcatcgagaccaaatttgagatgatcaaacttatagatattgcacgacagactgcccagggcatggattacttacacgccaagtcaatcatccacagagacctcaagagtaataatatatttcttcacgaagacctcacggttaaaataggtgattttggtctagccacagtgaaatctcgatggagtgggtcccatcagtttgaacagttgtctggatccattttgtggatggcaccagaagtaatcagaatgcgagataaaaacccatacagttttcagtccgatgtatatgcatttgggattgttctatatgaattgatgactgggcagttaccctattcaaatatcaacaacagggaccagataatttttatggtgggacgaggatatctatctccagatctcagcaaggtacggagtaactgtccaaaagccatgaagaggttaatggcggagtgcctcaaaaagaaaagagatgagagaccactctttccccaaattctcgcctctattgagctgctggcccgctcattgccaaaaattcaccgcagtgcatcagaaccctccttgaatcgggctggtttccaaacagaggattttagtctctatgcttgtgcttctccaaaaacacccatccaggcagggggatatggtgcgtttcctgtccactgatgcaaattaaatgagtgagaaataaa

SEQ ID NO: 10 - protein, 719 aa, Cavia porcellus
MAALSGGGGAEQGQALFNGDMELEAGAGAAASSAADPAIPEEVWNIKQMIKLTQEHIEALLDKFGGEHNPPSIYLEAYEEYTSKLDALQQREQQLLESLGNGTDFSVSSSASLDTVTSSSSSSLSVLPSSLSVFQNPTDVSRSNPKSPQKPIVRVFLPNKQRTVVPARCGVTVRDSLKKALMMRGLIPECCAVYRIQDGEKKPIGWDTDISWLTGEELHVEVLENVPLTTHNFVCIFIFFLLFVSKFFEHHPIPQEEASLAETTLTSGSSPSAPPSESIGPPILTSPSPSKSIPIPQPFRPGEEDHRNQFGQRDRSSSAPNVHINTIEPVNIDDLIRDQGFRSDGGSTTGLSATPPASLPGSLTNVKALQKSPGPQRERKSSSSSEDRNRMKTLGRRDSSDDWEIPDGQITVGQRIGSGSFGTVYKGKWHGDVAVKMLNVTAPTPQQLQAFKNEVGVLRKTRHVNILLFMGYSTKPQLAIVTQWCEGSSLYHHLHIIETKFEMIKLIDIARQTAQGMDYLHAKSIIHRDLKSNNIFLHEDLTVKIGDFGLATVKSRWSGSHQFEQLSGSILWMAPEVIRMRDKNPYSFQSDVYAFGIVLYELMTGQLPYSNINNRDQIIFMVGRGYLSPDLSKVRSNCPKAMKRLMAECLKKKRDERPLFPQILASIELLARSLPKIHRSASEPSLNRAGFQTEDFSLYACASPKTPIQAGGYGAFPVH

SEQ ID NO: 11 - DNA, 3229 bp, Canis familiaris
gtaatgctggattttcatggaataagtttgacctgtgctgcagtggcctccagcaaggtacccgcaagatgtggagttacagtccgggacagtctaaagaaagctctgatgatgagaggtctaatcccagagtgctgtgctgtttacagaattcaggatggagagaagaaaccgattggctgggacactgatatttcctggctcactggagaggaattgcatgtagaagtgttggaaaatgttccgcttaccacacacaactttgtacggaaaacttttttcaccttagcattttgtgacttttgtcgaaagctgcttttccagggttttcgctgtcaaacatgtggttataaatttcaccagcgttgtagtacagaggttccactgatgtgtgttaattatgaccaacttgatttgctgtttgtctccaagttctttgaacaccacccaataccacaggaggaggcctccatagcagagactgcccttacgtctggatcatccccttctgctcccccctccgattctcctgggcccccaattctgaccagtccgtctccttcaaaatccattccaattccacagcctttccgaccagcagatgaagatcatcgaaatcagtttggacaacgagaccggtcctcatcagctccaaatgtgcatataaacacaatagaacccgtcaacattgatgacttgattagagaccaagggtttcgtagtgatggaggatcaaccacaggtttgtctgccaccccccctgcctcattgcctggctcactcactaatgtaaaagcattacagaaatctccaggacctcagcgggaaagaaaatcatcttcatcctcagaagataggaatcgaatgaaaacacttggtagacgggattcaagtgatgattgggagatacctgatgggcagatcacagtgggacagagaattggatccgggtcatttgggacagtctacaagggaaagtggcatggtgacgtggcagtgaaaatgttgaatgtgacagcacccacacctcagcagttacaggccttcaaaaatgaagtaggagtactcaggaaaactcgacatgtgaatatcctactctttatgggctattcaacaaagccccaactggctattgttacccagtggtgtgagggctccagcttatatcaccatctccacatcattgagaccaaatttgagatgataaagcttatagatattgcacggcagactgcacagggcatggattacttacacgccaagtcaatcatccacagagacctcaagagtaataatatttttcttcatgaagacctcacagtaaaaataggtgattttggtctagccacagtgaaatctcgatggagtgggtcccatcagtttgaacagttgtctggatccattttgtggatggcaccagaagtgatccgaatgcaagacaaaaacccatatagcttccagtcagatgtatacgcatttgggattgttctatatgaattgatgacagggcagttaccttattcaaacatcaacaacagggaccagataatttttatggtgggacgaggatatctttctccagatctcagtaaggtacggagtaactgtccaaaagccatgaagagattgatggcagagtgcctaaaaaagaaaagagatgagaggccactctttccccaaattctcgcctctattgagctgctggcccgctcattgccaaaaattcaccgcagtgcatcagaaccctccttgaatcgggctggcttccaaacagaggattttagtctctatgcttgcgcttctccaaaaacacccatccaggcagggggatacggagaatttgcagccttcaagtagccacaccatcatggcaacaactactcttatttcttaagtcttgtgttcgtacaatttgttaacatcaaaacacagttctgttcctcaaatctttttttaaagatacagaattttcaatgcataagctggtgtggaacagaatggaatttcccatccaacaaaagagggaagaatgttttaggaaccagaattctctgctgccagtgtttcttcttcaacacaaataccacgtgcatacaagtctgcccactcccaggaaggaagaggagagcctgagttctgaccttttgatggtcaggcatgatggaaagaaactgctgctacagcttgggagattggctgtggagagcctgcccgtcagctctgcccttctaaccgccagatgagtgtgtggctggtcacctgacagggcagctgcaatcgccaagcatcgttctctttcctgtcctgggattttgtcgtggagctctttccccctagtcaccaccggttcatttctgagggatggaacaaaaatgcagcatggcctttctgtgtggtgcatgtccggtctttgacaaatttttatcaagtgaagctcttgtatttaaatggagaatgagaggcgagggggggggatcacgttttggtgtaggggcaaagggaatgctgcatctttttcctgacccactgggtttctggcctttgtttccttgctcactgagggtgtctgcctataaccacgcaggctggaaagtgctggcacacattgccttctcttctcactgggtccagcaatgaagacaagtgttggggatttttttttttgccctccacaatgtagcaagttctcaggaaaatacagttaatatcttcctcctaagctcttccagtcatcaagtacttatgtggctactttgtccagggcacaaaatgccatggcggtatccaattaaaagcctacaaaactgcttgataacagttttgaatgtgtgagacatttatgtaatttaaatgtaaggtacaagttttaatttctgagtttctctattatatttttattaaaaagaaaataattttcagatttaattgaattggaataaaataatacttcccaccagaattatatatcctggaaaattgtatttttgttatataaacaacttttaaagaaagatcattatccttttctctacctaaatatggggagtcttagcataatgacagatatttataatttttaaattaatggtacttgctggatccacactaacatctttgctaatatctcatgttttcctccaacttactcctacactacatcctccatcctctttccagtcttttatctagaatatgcaacctaaaataaaaatggtggtgtctccattca

SEQ ID NO: 12 - protein, 617 aa, Canis familiaris
MLDFHGISLTCAAVASSKVPARCGVTVRDSLKKALMMRGLIPECCAVYRIQDGEKKPIGWDTDISWLTGEELHVEVLENVPLTTHNFVRKTFFTLAFCDFCRKLLFQGFRCQTCGYKFHQRCSTEVPLMCVNYDQLDLLFVSKFFEHHPIPQEEASIAETALTSGSSPSAPPSDSPGPPILTSPSPSKSIPIPQPFRPADEDHRNQFGQRDRSSSAPNVHINTIEPVNIDDLIRDQGFRSDGGSTTGLSATPPASLPGSLTNVKALQKSPGPQRERKSSSSSEDRNRMKTLGRRDSSDDWEIPDGQITVGQRIGSGSFGTVYKGKWHGDVAVKMLNVTAPTPQQLQAFKNEVGVLRKTRHVNILLFMGYSTKPQLAIVTQWCEGSSLYHHLHIIETKFEMIKLIDIARQTAQGMDYLHAKSIIHRDLKSNNIFLHEDLTVKIGDFGLATVKSRWSGSHQFEQLSGSILWMAPEVIRMQDKNPYSFQSDVYAFGIVLYELMTGQLPYSNINNRDQIIFMVGRGYLSPDLSKVRSNCPKAMKRLMAECLKKKRDERPLFPQILASIELLARSLPKIHRSASEPSLNRAGFQTEDFSLYACASPKTPIQAGGYGEFAAFK

SEQ ID NO: 13 - DNA, 1889 bp, Canis familiaris
ggaatatcaaacaaatgattaagttgacacaggaacatatagaagccctattggacaagtttggtggggagcataatccaccatcaatatatctggaggcctatgaagaatacaccagcaaactagatgccctccaacagcgagaacaacagttattggaatccctggggaatggaactgatttttctgtttctagctctgcatcaacggacaccgttacatcttcttcctcttctagcctttcagtgctaccttcatctctttcagtttttcaaaatcccacagatatatcacggagcaatcccaagtcaccacaaaaacctatcgttagagtcttcctgcccaataaacagaggacggtggtacccgcaagatgtggagttacagtccgggacagtctaaagaaagctctgatgatgagaggtctaatcccagagtgctgtgctgtttacagaattcaggatggagagaagaaaccgattggctgggacactgatatttcctggctcactggagaggaattgcatgtagaagtgttggaaaatgttccgcttaccacacacaactttgtacggaaaacttttttcaccttagcattttgtgacttttgtcgaaagctgcttttccagggttttcgctgtcaaacatgtggttataaatttcaccagcgttgtagtacagaggttccactgatgtgtgttaattatgaccaacttgatttgctgtttgtctccaagttctttgaacaccacccaataccacaggaggaggcctccatagcagagactgcccttacgtctggatcatccccttctgctcccccctccgattctcctgggcccccaattctgaccagtccgtctccttcaaaatccattccaattccacagcctttccgaccagcagatgaagatcatcgaaatcagtttggacaacgagaccggtcctcatcagctccaaatgtgcatataaacacaatagaacccgtcaacattgatgacttgattagagaccaagggtttcgtagtgatggaggatcaaccacaggtttgtctgccaccccccctgcctcattgcctggctcactcactaatgtaaaagcattacagaaatctccaggacctcagcgggaaagaaaatcatcttcatcctcagaagataggaatcgaatgaaaacacttggtagacgggattcaagtgatgattgggagatacctgatgggcagatcacagtgggacagagaattggatccgggtcatttgggacagtctacaagggaaagtggcatggtgacgtggcagtgaaaatgttgaatgtgacagcacccacacctcagcagttacaggccttcaaaaatgaagtaggagtactcaggaaaactcgacatgtgaatatcctactctttatgggctattcaacaaagccccaactggctattgttacccagtggtgtgagggctccagcttatatcaccatctccacatcattgagaccaaatttgagatgataaagcttatagatattgcacggcagactgcacagggcatggattacttacacgccaagtcaatcatccacagagacctcaagagtaataatatttttcttcatgaagacctcacagtaaaaataggtgattttggtctagccacagtgaaatctcgatggagtgggtcccatcagtttgaacagttgtctggatccattttgtggatggcaccagaagtgatccgaatgcaagacaaaaacccatatagcttccagtcagatgtatacgcatttgggattgttctatatgaattgatgacagggcagttaccttattcaaacatcaacaacagggaccagctcagatcatgatcacggtgtcatgagatcaagccccac

SEQ ID NO: 14 - protein, 615 aa, Canis familiaris
MIKLTQEHIEALLDKFGGEHNPPSIYLEAYEEYTSKLDALQQREQQLLESLGNGTDFSVSSSASTDTVTSSSSSSLSVLPSSLSVFQNPTDISRSNPKSPQKPIVRVFLPNKQRTVVPARCGVTVRDSLKKALMMRGLIPECCAVYRIQDGEKKPIGWDTDISWLTGEELHVEVLENVPLTTHNFVRKTFFTLAFCDFCRKLLFQGFRCQTCGYKFHQRCSTEVPLMCVNYDQLDLLFVSKFFEHHPIPQEEASIAETALTSGSSPSAPPSDSPGPPILTSPSPSKSIPIPQPFRPADEDHRNQFGQRDRSSSAPNVHINTIEPVNIDDLIRDQGFRSDGGSTTGLSATPPASLPGSLTNVKALQKSPGPQRERKSSSSSEDRNRMKTLGRRDSSDDWEIPDGQITVGQRIGSGSFGTVYKGKWHGDVAVKMLNVTAPTPQQLQAFKNEVGVLRKTRHVNILLFMGYSTKPQLAIVTQWCEGSSLYHHLHIIETKFEMIKLIDIARQTAQGMDYLHAKSIIHRDLKSNNIFLHEDLTVKIGDFGLATVKSRWSGSHQFEQLSGSILWMAPEVIRMQDKNPYSFQSDVYAFGIVLYELMTGQLPYSNINNRDQLRS

SEQ ID NO: 15 - DNA, 3521 bp, Felis catus
  misc_feature (630)..(649): n is a, c, g, or t
atgcctaacctcagtctctgccaccacggccaatttgctcatgtgcccactgtgtcggcactgggatattttgtgatttgccttggccattgtccactgtccttgacattgcctgaaggagaaccactgatgctaatgttgaaggtgacctttgcaggctctccactactcataccaaagatgcggccccctgataatcccagagccactgtctgcacatgggcaaaacaggctacattctgtgcagactggggagaaaggttccaagaacacagtgccatagttttgggcagagagtttcaacacagcatagtgtctatggcagtatctggatttggccgggggaagtgcccaagaggagacagtcaggctgtgtcctacggccaaggacctgcacttatttttgcatgcagtggtttagcacagggaagagaacgaagtaggaaatcggagccatggaaacggcagagcggaggaaacgtgcacgcgcgagggtgggcacgaaaggaaagaaccctccccagaagactgcgcgagggcgctcctaggattacgtcacgcaccccgcgaaaactgaaatgtactgtgtgtggtcttttaattgaactatcttccttatgtgcacttaannnnnnnnnnnnnnnnnnnngcggcggcggcggtggcgcggagcagggccaggctctgttcaacggggacatggagcccgaagccggcgccgcggcctcttcggctgcggaccctgccattcccgaggaggtgtggaatatcaaacaaatgattaagttgacacaggaacatatagaggccctattggacaaatttggtggggagcataatccaccatcaatatatctagaggcctatgaagaatacaccagcaagctagatgccctccaacagagagaacaacagttattggaatccctggggaatggaactgatttttctgtttctagctctgcatcaacagacaccgttacatcttcctcctcttctagcctttcagtgctaccttcatctctttcagtttttcaaaaccccacagatgtgtcacggagcaatcccaagtcaccacagaaacctatcgttagagtcttcctgcctaataaacagaggacagtggtacctgcaagatgtggagttacagtccgggacagtctaaagaaagctctgatgatgagaggtctaatccctgagtgctgtgctgtttacagaattcaggatggagagaagaaaccaattggctgggacactgatatctcctggctcaccggagaggaattgcatgtagaagtgttggaaaatgttccacttacaactcacaactttgtatgtacggaaaacgttttcaccttagcattttgtgacttttgtcgaaagctgcttttccaaggttttcgctgtcaaacgtgtggttataaatttcaccagcgttgtagtacagaggttccactgatgtgtgttaattatgaccaacttgatttgctgtttgtctccaagttctttgaacaccacccaataccacaggaggaggcctccatagcagagactgccctaacgtctggatcgtccccttctgcccccccctccgattctactgggccccaaattctcaccagtccgtctccttcaaaatccattccaattccacagcctttccgaccagcagatgaagatcatcgaaatcaatttggacagcgagaccggtcctcatcagctccaaatgtgcatataaatacaatagaacctgtcaatattgatgacttgattagagaccaggggtttcgtagtgatggaggatcaaccacaggcttgtctgccaccccccctgcctcattgccgggctctctcactaatgtaaaagcattacagaaatctccagggcctcagcgggaaaggaaatcttcttcatcctcagaagataggaatcgaatgaaaacacttggtagaagggattcaagtgatgattgggagattcctgatgggcagatcacagtgggacagagaattggatccgggtcatttgggacagtctacaagggaaagtggcatggtgatgtggcagtgaaaatgttgaatgtgacagcacccacacctcagcagttacaggccttcaaaaatgaagtaggagtactcaggaaaactcggcatgtgaacatcctgctcttcatgggctattcaacaaagccccagctggctattgtcacccagtggtgtgagggctccagcttataccaccatctccacatcatcgagaccaaattcgagatgatcaagctgatagatattgctcggcagactgcgcagggcatggattacttacacgccaagtcaatcatccacagagacctcaagagtaataatatttttcttcacgaagacctcacagtaaaaataggtgattttggtctagccacagtgaaatctcgatggagtgggtcccatcagtttgaacagttgtctggatccattttgtggatggcaccagaagtaattcgaatgcaagataaaaacccatatagctttcagtcagatgtatatgcatttgggattgttctatatgaattgatgactggacagttaccttattcaaacatcaacaacagggaccagataatttttatggtgggacgaggatatctttctccagatctcagtaaggtacgaagtaactgtccaaaagccatgaagagattgatggcagagtgcctaaaaaagaaaagagatgagaggccactgtttccccaaattcttgcctctattgagctgctggcccgctcattgccaaaaattcaccgcagtgcatcagaaccctccttgaatcgggctggcttccagacagaggattttagtctctatgcttgtgcttctccaaaaacacccatccaggcagggggatatggtgcgtttcccgtccactgagataagttagatgagtgcgcgagtgcagggggccggggccaaggaggtggaaatgtgcgtgcttctgtactaagttggatagcatcttcttttttaaaaaaagatgaaccaaagaatgtgtatgtttttaaagactagatataattatttcctgatctaaaatgtatacttagctttggattttcaatatccaagggttttcaaaatgcacagacattgctgaacatttgcagtacctcttctggaggctttacttcctgttacaaattggttttgtttactggcttatcctaattattaaacttcaattaaacttttctcctgcaccttttgttatgagctatcacatgtcccttagggactcgcaagagcagtactgcccccgtgtacgggcttgcaggtagaaaggggatgacgggttttaacacctgtgtgaggcaaggcagtccgaacagatctcatttaggaagccacgagagttgaataagttatttttattcttagtattttttctgtaactactttttattataacttggaaaatatggatgtcctttatacaccttagcaatagactgaatttctttttataaatt

SEQ ID NO: 16 - protein, 974 aa, Felis catus
  misc_feature (210)..(217): Xaa can be any naturally occurring amino acid
MPNLSLCHHGQFAHVPTVSALGYFVICLGHCPLSLTLPEGEPLMLMLKVTFAGSPLLIPKMRPPDNPRATVCTWAKQATFCADWGERFQEHSAIVLGREFQHSIVSMAVSGFGRGKCPRGDSQAVSYGQGPALIFACSGLAQGRERSRKSEPWKRQSGGNVHARGWARKERTLPRRLREGAPRITSRTPRKLKCTVCGLLIELSSLCALXXXXXXXXGGGGGAEQGQALFNGDMEPEAGAAASSAADPAIPEEVWNIKQMIKLTQEHIEALLDKFGGEHNPPSIYLEAYEEYTSKLDALQQREQQLLESLGNGTDFSVSSSASTDTVTSSSSSSLSVLPSSLSVFQNPTDVSRSNPKSPQKPIVRVFLPNKQRTVVPARCGVTVRDSLKKALMMRGLIPECCAVYRIQDGEKKPIGWDTDISWLTGEELHVEVLENVPLTTHNFVCTENVFTLAFCDFCRKLLFQGFRCQTCGYKFHQRCSTEVPLMCVNYDQLDLLFVSKFFEHHPIPQEEASIAETALTSGSSPSAPPSDSTGPQILTSPSPSKSIPIPQPFRPADEDHRNQFGQRDRSSSAPNVHINTIEPVNIDDLIRDQGFRSDGGSTTGLSATPPASLPGSLTNVKALQKSPGPQRERKSSSSSEDRNRMKTLGRRDSSDDWEIPDGQITVGQRIGSGSFGTVYKGKWHGDVAVKMLNVTAPTPQQLQAFKNEVGVLRKTRHVNILLFMGYSTKPQLAIVTQWCEGSSLYHHLHIIETKFEMIKLIDIARQTAQGMDYLHAKSIIHRDLKSNNIFLHEDLTVKIGDFGLATVKSRWSGSHQFEQLSGSILWMAPEVIRMQDKNPYSFQSDVYAFGIVLYELMTGQLPYSNINNRDQIIFMVGRGYLSPDLSKVRSNCPKAMKRLMAECLKKKRDERPLFPQILASIELLARSLPKIHRSASEPSLNRAGFQTEDFSLYACASPKTPIQAGGYGAFPVH

SEQ ID NO: 17 - DNA, 3853 bp, Bos taurus
ctcagctgcgccgggtctcacaagacggttcccgaggtggcccaggcgccgtcccaccgccgacgccgcccgggccgcccgggccgtccctccccgctgccccccgtcctccgcctccgcctccccccgccctcagcctcccttccccctccccgcccagcagcggtcgctcgggcccggctctcggttataagatggcggcgctgagtggcggcggcggcggcggcggcggtggcgcggagcagggccaggctctgttcaacggggacatggagcccgaggccggcgccgcggcctcttcggctgcggaccccgccattcccgaggaggtgtggaatatcaaacaaatgattaagttgacacaggagcatatagaggccctattggacaaatttggtggggagcataatccaccatcaatatatctggaggcctatgaagaatacaccagcaagctagatgccctccaacaaagagaacaacagttattggaatccctggggaatggaactgatttttctgtttctagctctgcatcaacggacaccgttacatcttcttcctcttctagcctttcagtgctgccttcatctctttcagtttttcaaaatcccacagatgtgtcacggagcaaccccaagtcaccacaaaaacctatcgttagagtcttcctgcccaataaacagaggacagtggtacctgcacggtgtggagtcacagtccgggacagcctgaagaaggcactgatgatgagaggtctaatcccagagtgctgtgctgtttacagaattcaggatggggagaagaaaccaattggctgggacactgatatttcctggcttactggagaggagttgcatgtagaagtgttggagaatgttccacttacaacacacaactttgtacggaaaacttttttcaccttagcattttgtgacttctgtagaaagctgcttttccagggattccgctgtcaaacatgtggttataaatttcaccagcgttgtagtacagaggttccactgatgtgtgttaattatgaccaactagatttgctgtttgtctccaagttctttgaacaccacccaataccacaggaggaggcctccttagcagagactacccttccatgtggctcatccccttctgcacccccctccgattctattgggcccccaattctcaccagtccatctccttcaaaatccattccaattccacagcctttccgaccagcagatgaagatcatcgaaatcagtttggacaacgagaccggtcctcatcagctccaaatgtgcatataaacacaatagaacccgtcaatattgatgacttgattagagaccaagggtttcgtagtgatggaggatcaaccacaggtttatccgccacaccccctgcctcattacctggctcactctctaatgtgaaagcattgcagaaatctccaggacctcagcgagaaagaaagtcctcttcatcctcagaagacaggaatcgaatgaaaacgcttggtagacgggattcaagtgacgattgggagattcctgatggacagatcacagtgggacaaagaattggatcagggtcatttgggacagtctacaagggaaagtggcatggtgatgtggcagtgaaaatgttgaatgtgacagcacccacacctcagcagttacaggccttcaaaaatgaagtaggagtactcaggaaaacgcgacatgtgaatatcctcctcttcatgggttattcaacaaagccacaactggctattgttacccagtggtgtgagggctccagtttatatcatcatctccacatcattgagaccaaattcgagatgatcaaacttatagatattgcacggcagactgcacagggcatggattacttacacgccaagtcaatcatccacagagacctcaagagtaataatatttttcttcatgaagacctcacagtaaaaataggtgattttggtctagccacagtgaaatctcgatggagtgggtcccatcagtttgaacagttgtctggatccattttgtggatggcaccagaagtaatcagaatgcaagataaaaacccatatagctttcagtcagatgtatatgcatttgggattgttctgtatgaattgatgaccggacagttaccttattcaaatatcaacaacagggaccagataatttttatggtgggacgaggatatctgtctccagatctcagtaaggtacggagtaactgtccaaaagccatgaagagattaatggcagagtgcctaaaaaagaaaagagatgaaagaccactctttccccaaattctcgcctctattgagctgctggcccgctcattgccaaaaattcaccgcagtgcatcagaaccctccttgaatcgggctggcttccaaacagaggattttagtctatatgcttgtgcttctccaaaaacacccattcaggcagggggatatggtacgtttcctgttcactgaaacaaaccgagtgagtgacagcatgtaggagggtagggacaaaagaaagtgaacaaatgtttgcttatatatttgttaaattgaataggattttctttttctttaaaggtgaacaagagaacatgtgtgtttttaaagtttggatatagttttcttcccagtctaaaacccatagttagcattacattttcaacatcgaatttttttttaattcatagacattgctgaaaatttataataccttttccagaggctttacttcccattccaagtttgttttgtttacttggttagtctaatcattaaactttaaactttccccacctaccttttgctgttagctatcccgcatccattaggggctccaagaacagcactgtctgcgtgtgtgtgttggcaggtgggaagctgatggtaagttaggctgtgttagtgaaggtaaactgaccaggtctaattaggagtcactagaattgaataagcttatttttattaatattttttcttataactatttctttttgtaataatttagaaaatataattgttctttattcccttacagcagtataaattattggtgcaggtaaccaaagatattactgaggagtggcatgtttgacatgagtgacatggtttaactttggatttttagttaatatttctttatatattaaggatgtcttacacattatagaagtcaaatttactgacaaaggtattgcctcctcttcctccccaaaaacacagcaaaattctctgggaactcgtagcattgttggttttcttttggatgactatggttgccaaacaaccaagtaattgattttttttaaattattattgctttagattatactcacctctcatgatgcctgttagcaatcacctttatccatgtgtcttgtaaaatatctttcctccttatattctttgcccaacaagagtctacttgttatgaatgagtactattttctttttttgattccccagtataattagtatgtttagtgctttctaggacttccactttcttatgttaaaaaaaaaaacaaactaatgtggcagtcagtatattcttactgtgaatcagagtctttactgggaatcaaagtgaaagaagcagctgttctgacttcagagtcagcctagggaccaaaaccagcctcttaaatacaccttcatttattcagtttggatttgtgatgattttcattatagctgacagttcaaggttattcagtggcacacagatagcatctgcataaatgcctttcttcttgaaaataaaggagaaaattgggaagactttacaccaatagtttagtctttaagtaccacagataacacacaccataaat

SEQ ID NO: 18 - protein, 764 aa, Bos taurus
AALSGGGGGGGGGAEQGQALFNGDMEPEAGAAASSAADPAIPEEVWNIKQMIKLTQEHIEALLDKFGGEHNPPSIYLEAYEEYTSKLDALQQREQQLLESLGNGTDFSVSSSASTDTVTSSSSSSLSVLPSSLSVFQNPTDVSRSNPKSPQKPIVRVFLPNKQRTVVPARCGVTVRDSLKKALMMRGLIPECCAVYRIQDGEKKPIGWDTDISWLTGEELHVEVLENVPLTTHNFVRKTFFTLAFCDFCRKLLFQGFRCQTCGYKFHQRCSTEVPLMCVNYDQLDLLFVSKFFEHHPIPQEEASLAETTLPCGSSPSAPPSDSIGPPILTSPSPSKSIPIPQPFRPADEDHRNQFGQRDRSSSAPNVHINTIEPVNIDDLIRDQGFRSDGGSTTGLSATPPASLPGSLSNVKALQKSPGPQRERKSSSSSEDRNRMKTLGRRDSSDDWEIPDGQITVGQRIGSGSFGTVYKGKWHGDVAVKMLNVTAPTPQQLQAFKNEVGVLRKTRHVNILLFMGYSTKPQLAIVTQWCEGSSLYHHLHIIETKFEMIKLIDIARQTAQGMDYLHAKSIIHRDLKSNNIFLHEDLTVKIGDFGLATVKSRWSGSHQFEQLSGSILWMAPEVIRMQDKNPYSFQSDVYAFGIVLYELMTGQLPYSNINNRDQIIFMVGRGYLSPDLSKVRSNCPKAMKRLMAECLKKKRDERPLFPQILASIELLARSLPKIHRSASEPSLNRAGFQTEDFSLYACASPKTPIQAGGYGTFPVH

SEQ ID NO: 19 - DNA, 4936 bp, Bos taurus
ctcagctgcgccgggtctcacaagacggttcccgaggtggcccaggcgccgtcccaccgccgacgccgcccgggccgcccgggccgtccctccccgctgccccccgtcctccgcctccgcctccccccgccctcagcctcccttccccctccccgcccagcagcggtcgctcgggcccggctctcggttataagatggcggcgctgagtggcggcggcggcggcggcggcggtggcgcggagcagggccaggctctgttcaacggggacatggagcccgaggccggcgccgcggcctcttcggctgcggaccccgccattcccgaggaggtgtggaatatcaaacaaatgattaagttgacacaggagcatatagaggccctattggacaaatttggtggggagcataatccaccatcaatatatctggaggcctatgaagaatacaccagcaagctagatgccctccaacaaagagaacaacagttattggaatccctggggaatggaactgatttttctgtttctagctctgcatcaacggacaccgttacatcttcttcctcttctagcctttcagtgctgccttcatctctttcagtttttcaaaatcccacagatgtgtcacggagcaaccccaagtcaccacaaaaacctatcgttagagtcttcctgcccaataaacagaggacagtggtacctgcacggtgtggagtcacagtccgggacagcctgaagaaggcactgatgatgagaggtctaatcccagagtgctgtgctgtttacagaattcaggatggggagaagaaaccaattggctgggacactgatatttcctggcttactggagaggagttgcatgtagaagtgttggagaatgttccacttacaacacacaactttgtacggaaaacttttttcaccttagcattttgtgacttctgtagaaagctgcttttccagggattccgctgtcaaacatgtggttataaatttcaccagcgttgtagtacagaggttccactgatgtgtgttaattatgaccaactagatttgctgtttgtctccaagttctttgaacaccacccaataccacaggaggaggcctccttagcagagactacccttccatgtggctcatccccttctgcacccccctccgattctattgggcccccaattctcaccagtccatctccttcaaaatccattccaattccacagcctttccgaccagcagatgaagatcatcgaaatcagtttggacaacgagaccggtcctcatcagctccaaatgtgcatataaacacaatagaacccgtcaatattgatgacttgattagagaccaagggtttcgtagtgatggaggatcaaccacaggtttatccgccacaccccctgcctcattacctggctcactctctaatgtgaaagcattgcagaaatctccaggacctcagcgagaaagaaagtcctcttcatcctcagaagacaggaatcgaatgaaaacgcttggtagacgggattcaagtgacgattgggagattcctgatggacagatcacagtgggacaaagaattggatcagggtcatttgggacagtctacaagggaaagtggcatggtgatgtggcagtgaaaatgttgaatgtgacagcacccacacctcagcagttacaggccttcaaaaatgaagtaggagtactcaggaaaacgcgacatgtgaatatcctcctcttcatgggttattcaacaaagccacaactggctattgttacccagtggtgtgagggctccagtttatatcatcatctccacatcattgagaccaaattcgagatgatcaaacttatagatattgcacggcagactgcacagggcatggattacttacacgccaagtcaatcatccacagagacctcaagagtaataatatttttcttcatgaagacctcacagtaaaaataggtgattttggtctagccacagtgaaatctcgatggagtgggtcccatcagtttgaacagttgtctggatccattttgtggatggcaccagaagtaatcagaatgcaagataaaaacccatatagctttcagtcagatgtatatgcatttgggattgttctgtatgaattgatgaccggacagttaccttattcaaatatcaacaacagggaccagataatttttatggtgggacgaggatatctgtctccagatctcagtaaggtacggagtaactgtccaaaagccatgaagagattaatggcagagtgcctaaaaaagaaaagagatgaaagaccactctttccccaagtaggaaagactctcctaagcaagagacaaaattcagaagttatcagggaaaaagataagcagattctcgcctctattgagctgctggcccgctcattgccaaaaattcaccgcagtgcatcagaaccctccttgaatcgggctggcttccaaacagaggattttagtctatatgcttgtgcttctccaaaaacacccattcaggcagggggatatgaagcagatttggctcttacatcaaataaaaatagagtagaagttgggatttagagatttcctgacatgcaagaaggaataagcaagaaaaaaaggtttgttttccccaaatcatatctattgtcttttacttctattttttcttaaattttttgtgatttcagagacatgtagagttttattgatacctaaactatgagttcttttttttttttttttttcattattttgatttttttggccaagaggcatatgggatcttagcttgagaaagcaacaattttcttgatgtcattttgggtgagggcacatattgctgtgaacagtgtggtgatagccaccagggaccaaactcacacccgctgcattgaaaggtgaagtcttaaacactggaccagcagagaaattcctactctatgagttctttttgtcatcccctccccgcaccctccacccccaacctaaagtctgatgatgaaatcaacaactattccattagaagcagtagattctggtagcatgatctttagtttgttagtaagattttgtgctttgtggggttgtgtcgttttaaggctaatatttaagtttgtcaaatagaatgctgttcagattgtaaaaatgagtaataaacatctgaagttttttttaagttatttttaacatggtatatacagttgagcttagagtttatcattttctgatattctcttacttagtagatgaattctagccattttttataaagatttctgttaagcaaatcctgttttcacatgggcttcctttaagggattttagattctgctggatatggtgactgctcataagactgttgaaaattacttttaagatgtattagaatacttctgaaaaaaaatagcaaccttaaaaccataagcaaaagtagtaagggtgtttatacatttctagagtccctgtttaggtaatagcctcctatgattgtactttaaatgttttgctctccaaggttttagtaacttggctttttttctaatcagtgccaaactcccccagtttttttaactttaaatatgaggtaataaatcttttacccttccttgatcttttgacttataataccttggtcagttgtttcttaaaaggaatccttaaatggaaagagacaatatcactgtctgcagttctgattagtagttttattcagaatggaaaaacagattattcatttttgaaaattgttcaggggtatgttcattgttaggaccttggactttggagtcagtgcctagctatgcattccaggtctgccattttctggctgtgaaattttggacaagttacttaaccactttaaaccccagctttaagaagtaaattaaccccagtaaattaagaagtaatagcagccacttcgtagagttgttatgaggctcagatgcagtgcaaatgtgtataaagtattcagggagtcacctggtatactataatagacactagaatagttgccaatattatcagcatacaatctgaggattctgtcagccaatcattagcaatctgttgtttgttgggacatgccagtgttctccagttgaaatcagtagcaatctaaaaatggatagattattcctcatttaaatagtgtgttcatataagtgattgcttggatccttatcagaagttgctgttactgaaaaatgataaggctgactaaattgtgatagttgtcagttactaaccaactcccagaaatgaataagaggaacctatctctagttcctagtagaaggtatggacaaaatagtaggtgaaaaataatgtcttgaacccccaaattaagtaagctttaaagagtacaatacctcaaagggtctttgcggtttaaaatttgtatgctgagaatgatgttcattgacatgtgcctatatgtaattttttgatagtttaaaaggtgaaatgaactacagatgggagaggtctgaattttcttgccttcagtcaaatgtgtaatgtggacatattatttgacctgtgaattttatcttttaaaaaagattaattcctgcttcttccttcctaatagttgcattataataatgaaaatgagttgataatttggggggaaagtattctacaaatcaaccttattattttaccattggtttctgagaaattttgttcatttgaaccgtttatagcttgattagaatcatagcatgtaaaacccaactgagggattatctgcagacttaatgtagtattatgtaagttgtcttctttcatttcgaccttttttgcttttgttgttgctagatctgtagtatgtagctagtcacctttcagcgaggtttcagcgaggcttttctgtgtctctaggttatttgagataacttttttaaaattagctcttgtcctcc

SEQ ID NO: 20 - protein, 797 aa, Bos taurus
MAALSGGGGGGGGGAEQGQALFNGDMEPEAGAAASSAADPAIPEEVWNIKQMIKLTQEHIEALLDKFGGEHNPPSIYLEAYEEYTSKLDALQQREQQLLESLGNGTDFSVSSSASTDTVTSSSSSSLSVLPSSLSVFQNPTDVSRSNPKSPQKPIVRVFLPNKQRTVVPARCGVTVRDSLKKALMMRGLIPECCAVYRIQDGEKKPIGWDTDISWLTGEELHVEVLENVPLTTHNFVRKTFFTLAFCDFCRKLLFQGFRCQTCGYKFHQRCSTEVPLMCVNYDQLDLLFVSKFFEHHPIPQEEASLAETTLPCGSSPSAPPSDSIGPPILTSPSPSKSIPIPQPFRPADEDHRNQFGQRDRSSSAPNVHINTIEPVNIDDLIRDQGFRSDGGSTTGLSATPPASLPGSLSNVKALQKSPGPQRERKSSSSSEDRNRMKTLGRRDSSDDWEIPDGQITVGQRIGSGSFGTVYKGKWHGDVAVKMLNVTAPTPQQLQAFKNEVGVLRKTRHVNILLFMGYSTKPQLAIVTQWCEGSSLYHHLHIIETKFEMIKLIDIARQTAQGMDYLHAKSIIHRDLKSNNIFLHEDLTVKIGDFGLATVKSRWSGSHQFEQLSGSILWMAPEVIRMQDKNPYSFQSDVYAFGIVLYELMTGQLPYSNINNRDQIIFMVGRGYLSPDLSKVRSNCPKAMKRLMAECLKKKRDERPLFPQVGKTLLSKRQNSEVIREKDKQILASIELLARSLPKIHRSASEPSLNRAGFQTEDFSLYACASPKTPIQAGGYEADLALTSNKNRVEVGI

SEQ ID NO: 21 - DNA, 4154 bp, Bos taurus
ctcagctgcgccgggtctcacaagacggttcccgaggtggcccaggcgccgtcccaccgccgacgccgcccgggccgcccgggccgtccctccccgctgccccccgtcctccgcctccgcctccccccgccctcagcctcccttccccctccccgcccagcagcggtcgctcgggcccggctctcggttataagatggcggcgctgagtggcggcggcggcggcggcggcggtggcgcggagcagggccaggctctgttcaacggggacatggagcccgaggccggcgccgcggcctcttcggctgcggaccccgccattcccgaggaggtgtggaatatcaaacaaatgattaagttgacacaggagcatatagaggccctattggacaaatttggtggggagcataatccaccatcaatatatctggaggcctatgaagaatacaccagcaagctagatgccctccaacaaagagaacaacagttattggaatccctggggaatggaactgatttttctgtttctagctctgcatcaacggacaccgttacatcttcttcctcttctagcctttcagtgctgccttcatctctttcagtttttcaaaatcccacagatgtgtcacggagcaaccccaagtcaccacaaaaacctatcgttagagtcttcctgcccaataaacagaggacagtggtacctgcacggtgtggagtcacagtccgggacagcctgaagaaggcactgatgatgagaggtctaatcccagagtgctgtgctgtttacagaattcaggatggggagaagaaaccaattggctgggacactgatatttcctggcttactggagaggagttgcatgtagaagtgttggagaatgttccacttacaacacacaactttgtacggaaaacttttttcaccttagcattttgtgacttctgtagaaagctgcttttccagggattccgctgtcaaacatgtggttataaatttcaccagcgttgtagtacagaggttccactgatgtgtgttaattatgaccaactagatttgctgtttgtctccaagttctttgaacaccacccaataccacaggaggaggcctccttagcagagactacccttccatgtggctcatccccttctgcacccccctccgattctattgggcccccaattctcaccagtccatctccttcaaaatccattccaattccacagcctttccgaccagcagatgaagatcatcgaaatcagtttggacaacgagaccggtcctcatcagctccaaatgtgcatataaacacaatagaacccgtcaatattgatgacttgattagagaccaagggtttcgtagtgatggaggatcaaccacaggtttatccgccacaccccctgcctcattacctggctcactctctaatgtgaaagcattgcagaaatctccaggacctcagcgagaaagaaagtcctcttcatcctcagaagacaggaatcgaatgaaaacgcttggtagacgggattcaagtgacgattgggagattcctgatggacagatcacagtgggacaaagaattggatcagggtcatttgggacagtctacaagggaaagtggcatggtgatgtggcagtgaaaatgttgaatgtgacagcacccacacctcagcagttacaggccttcaaaaatgaagtaggagtactcaggaaaacgcgacatgtgaatatcctcctcttcatgggttattcaacaaagccacaactggctattgttacccagtggtgtgagggctccagtttatatcatcatctccacatcattgagaccaaattcgagatgatcaaacttatagatattgcacggcagactgcacagggcatggattacttacacgccaagtcaatcatccacagagacctcaagagtaataatatttttcttcatgaagacctcacagtaaaaataggtgattttggtctagccacagtgaaatctcgatggagtgggtcccatcagtttgaacagttgtctggatccattttgtggatggcaccagaagtaatcagaatgcaagataaaaacccatatagctttcagtcagatgtatatgcatttgggattgttctgtatgaattgatgaccggacagttaccttattcaaatatcaacaacagggaccagataatttttatggtgggacgaggatatctgtctccagatctcagtaaggtacggagtaactgtccaaaagccatgaagagattaatggcagagtgcctaaaaaagaaaagagatgaaagaccactctttccccaagtaggaaagactctcctaagcaagagacaaaattcagaagttatcagggaaaaagataagcagattctcgcctctattgagctgctggcccgctcattgccaaaaattcaccgcagtgcatcagaaccctccttgaatcgggctggcttccaaacagaggattttagtctatatgcttgtgcttctccaaaaacacccattcaggcagggggatatggctgagcacattgtccatcacccacaagtggctggttctcatcgcagaatctacgtagggaatcgggcgtgaaattcacttaagagatagagcagaggaagtgttctgtttacaggaatggagatgagagttatgagtaagttgcttagtcagttggctttgttttgaaaattattgtgttatatttgtgttaacctacttgtgttttgacagtatatgtcacataggaagaaacctcagactagcataataacaaagctcagactaggcacagatgtacacagaatggaccaaaatgggatgggggaaggtatgggaataagtctaggggtagggaaaaattgatgtgagggtgggaaataaactgtaattacctgaaataaaatgtaagagtgcaataagtgtgctttttattctaagctgtgaatgggttttttaaaaaaagcattccttcccaatgcatttgcctatgttccatagctgattaaaaccagctatataaacatatgcctttttattcatgttaattaccaatataaatggctaacctttacgtcttatttatcttcatgttatgttagtttacatacagggatgtgtgtgtgtgtgtatgctataaattttccctccttcgtttaaaaacgcgtttgttggatcctctctgtttccttaggccatgccacagctcatagtctcagcttggccttcctgtcacctgatctgaaggactatcacagtgacgtagctcgttcattggttgtacacactctaacccttttccttgctcagcaattactgtgtcttctaaaacaggagtgtacaaccatgagattgcaattaattgtttgacatatgtccctttgaattctatttattagttatgattgattgctctttggtttggaccaagaaaaacgaaatcccacctccccaccttttcacttatttcttactttgaggacaattctgtaagagagaggaaagggaactccttcatgttttaactgcagcaagttaatggccctggtttacaccaaacattatggtgattcacattcacattcctctcctctcttgctgccagaggtttgggttttgttcagttctgctcaagcactgaaaaagttttcatggagtctggagagtgcccagtgaaaagatggtttttaattgtccacagacctttctgttcctgctttgcaaaaattacaaaggagtaactatttttaaagcttatttttcaattcataaaaaagacatttattttcagtcagatgatgtctccttgtcccttaatcctcaatgtttgcttgaatcttttttttttttctgattttctcccatccccacttcttgatacttcttgagttctctttcctgctcaggtcctttcatttgtactttggagttttttctcatgtaaatttgtacaatggaaaatattgttcagtttggatagaacgcatggagaattaaataaaaaagatagctgaaattcagattgaaatttatttgtgtaaagttatttaaaaactctgtactatataaaaggcaaaaaaagttctatgtacttgatgtgaatatgcgaatactgctataataaagattgactgcatgga

SEQ ID NO: 22 - protein, 781 aa, Bos taurus
MAALSGGGGGGGGGAEQGQALFNGDMEPEAGAAASSAADPAIPEEVWNIKQMIKLTQEHIEALLDKFGGEHNPPSIYLEAYEEYTSKLDALQQREQQLLESLGNGTDFSVSSSASTDTVTSSSSSSLSVLPSSLSVFQNPTDVSRSNPKSPQKPIVRVFLPNKQRTVVPARCGVTVRDSLKKALMMRGLIPECCAVYRIQDGEKKPIGWDTDISWLTGEELHVEVLENVPLTTHNFVRKTFFTLAFCDFCRKLLFQGFRCQTCGYKFHQRCSTEVPLMCVNYDQLDLLFVSKFFEHHPIPQEEASLAETTLPCGSSPSAPPSDSIGPPILTSPSPSKSIPIPQPFRPADEDHRNQFGQRDRSSSAPNVHINTIEPVNIDDLIRDQGFRSDGGSTTGLSATPPASLPGSLSNVKALQKSPGPQRERKSSSSSEDRNRMKTLGRRDSSDDWEIPDGQITVGQRIGSGSFGTVYKGKWHGDVAVKMLNVTAPTPQQLQAFKNEVGVLRKTRHVNILLFMGYSTKPQLAIVTQWCEGSSLYHHLHIIETKFEMIKLIDIARQTAQGMDYLHAKSIIHRDLKSNNIFLHEDLTVKIGDFGLATVKSRWSGSHQFEQLSGSILWMAPEVIRMQDKNPYSFQSDVYAFGIVLYELMTGQLPYSNINNRDQIIFMVGRGYLSPDLSKVRSNCPKAMKRLMAECLKKKRDERPLFPQVGKTLLSKRQNSEVIREKDKQILASIELLARSLPKIHRSASEPSLNRAGFQTEDFSLYACASPKTPIQAGGYG

SEQ ID NO: 23 - DNA, 7914 bp, Bos taurus
ctcagctgcgccgggtctcacaagacggttcccgaggtggcccaggcgccgtcccaccgccgacgccgcccgggccgcccgggccgtccctccccgctgccccccgtcctccgcctccgcctccccccgccctcagcctcccttccccctccccgcccagcagcggtcgctcgggcccggctctcggttataagatggcggcgctgagtggcggcggcggcggcggcggcggtggcgcggagcagggccaggctctgttcaacggggacatggagcccgaggccggcgccgcggcctcttcggctgcggaccccgccattcccgaggaggtgtggaatatcaaacaaatgattaagttgacacaggagcatatagaggccctattggacaaatttggtggggagcataatccaccatcaatatatctggaggcctatgaagaatacaccagcaagctagatgccctccaacaaagagaacaacagttattggaatccctggggaatggaactgatttttctgtttctagctctgcatcaacggacaccgttacatcttcttcctcttctagcctttcagtgctgccttcatctctttcagtttttcaaaatcccacagatgtgtcacggagcaaccccaagtcaccacaaaaacctatcgttagagtcttcctgcccaataaacagaggacagtggtacctgcacggtgtggagtcacagtccgggacagcctgaagaaggcactgatgatgagaggtctaatcccagagtgctgtgctgtttacagaattcaggatggggagaagaaaccaattggctgggacactgatatttcctggcttactggagaggagttgcatgtagaagtgttggagaatgttccacttacaacacacaactttgtacggaaaacttttttcaccttagcattttgtgacttctgtagaaagctgcttttccagggattccgctgtcaaacatgtggttataaatttcaccagcgttgtagtacagaggttccactgatgtgtgttaattatgaccaactagatttgctgtttgtctccaagttctttgaacaccacccaataccacaggaggaggcctccttagcagagactacccttccatgtggctcatccccttctgcacccccctccgattctattgggcccccaattctcaccagtccatctccttcaaaatccattccaattccacagcctttccgaccagcagatgaagatcatcgaaatcagtttggacaacgagaccggtcctcatcagctccaaatgtgcatataaacacaatagaacccgtcaatattgatgacttgattagagaccaagggtttcgtagtgatggaggatcaaccacaggtttatccgccacaccccctgcctcattacctggctcactctctaatgtgaaagcattgcagaaatctccaggacctcagcgagaaagaaagtcctcttcatcctcagaagacaggaatcgaatgaaaacgcttggtagacgggattcaagtgacgattgggagattcctgatggacagatcacagtgggacaaagaattggatcagggtcatttgggacagtctacaagggaaagtggcatggtgatgtggcagtgaaaatgttgaatgtgacagcacccacacctcagcagttacaggccttcaaaaatgaagtaggagtactcaggaaaacgcgacatgtgaatatcctcctcttcatgggttattcaacaaagccacaactggctattgttacccagtggtgtgagggctccagtttatatcatcatctccacatcattgagaccaaattcgagatgatcaaacttatagatattgcacggcagactgcacagggcatggattacttacacgccaagtcaatcatccacagagacctcaagagtaataatatttttcttcatgaagacctcacagtaaaaataggtgattttggtctagccacagtgaaatctcgatggagtgggtcccatcagtttgaacagttgtctggatccattttgtggatggcaccagaagtaatcagaatgcaagataaaaacccatatagctttcagtcagatgtatatgcatttgggattgttctgtatgaattgatgaccggacagttaccttattcaaatatcaacaacagggaccagataatttttatggtgggacgaggatatctgtctccagatctcagtaaggtacggagtaactgtccaaaagccatgaagagattaatggcagagtgcctaaaaaagaaaagagatgaaagaccactctttccccaaattctcgcctctattgagctgctggcccgctcattgccaaaaattcaccgcagtgcatcagaaccctccttgaatcgggctggcttccaaacagaggattttagtctatatgcttgtgcttctccaaaaacacccattcaggcagggggatatggagaatttgcagccttcaagtagccacaccatcatgacagcatctactcttatttcttaagtcttgtgttcgtacaatttgttaacatcaaaacacagttctgttcctcaactctttttaaagttaaaatttttcagtgcataagctggtgtggaacagaaggaaatttcccatccaacaaaagagggaagaatgttttaggaaccagaattctctgctgccagtgtttcttcttcaacacaaatatcacaagtctgcccactcccaggaagaaagaggagagaccctgagttctgaccttttgatggtcaggcatgatggaaagaaactgctgctacagcttgggagatttgctctgggaagtctgccagtcaactttgcccttctaaccaccagatcaatatgtggctgatcatctgatggggcagttgcaatcaccaagccttgttctctttcctgttctgggattgtgttgtggaacccttttccctagccaccaccagttcatttctgagggatggaacaaaaatgcagcatgcccttcctgtgtggtgcatgttcagtccttgacaaatttttaccaaaatgaagctactttatttaaaaggagggtgagaggtgaggaggtcactttgggtgtggcggaaagggaatgctgcatctttttcctgggctgctggggctctggccttggcttgccagccggaagcgctggcacgcatcgccttcttttcccattgggtccagcaatgaagacgagtgtttggggttttttttttctccaccatgtagcaagttctcaggaaaatacaattgatatcttcctcctaagctcttccaatcagtcaccaagtacttatgtggttactttgtccagggcacaaaatgcctgtatctaattaaaagcctacaaaactgcttgataacagttttgaatgtgagacatttatgtaatttaaatgtaaggtacaagttttaatttctgagtttcttctattatatttttattaaaaaaagaaaataattttcagattgaattggagtaaaataatattacttcccactagaattatatatcctggaaaattgtatttttgttacataagcagcttttaaagaaagatcattacccttttctctacataaatatatggggagtcttagcctaatgacaaatatttataatttttaaattaatggtacttgctggatccatactaacatctttactaatacctcattgtttcttccaacttactcctacactacatcctacatcttcttcctagtcttttatctagaatatgcaacctcaaataaaaatggtggtgtcctcattcattctcctccttccttttttcccaagcctgatcttcaaaaggttggttaatttggcagctgagttcctccccaggcagagaatagaccaattttaggtgtattgggactgagggaggatgtgtaaagattaacatcagtaaagaaccgctgtggagtaattaagaactttgttctttataactggagaatataacctaaccctaacatccctcagcctttactaaagtgtggcgtaaatcacagtagtagcaaagaaagtgactctggatgtgttcctggccagtacctcccttatcatgaatgtagactctctcatcaagatttaggaatataaatcaaatcaaatgtgcccagccaagctatgtagtaagggacttgaacaatattaggcagaacctataaaataaatcagggaattagaaattatttaaagttttcaaattgtaaattgccccggtgtctttcagcctactgccattatttttgctacaatacctacatttcagaggagggcctactgaaaattccatgcaagtggaaaataatcctcaagttattaatgagtttgaaaagcaatgagttcttaagtctttgtgagtagagcaagatcctacaaaattcagaaatagtaaaaatggattcatgctgatttgaagagcatctgtgtgcataatataatgctgcatctcttttaaaagcagtctatttttctttttaaatttgtccccatagatgcttttgaacatgaacatgcttatgttaccttttccgaggttgggaagagccaggagctctcaggcagggccccctccctcagctgggcaggagctgctcaggaggagctagttatagaggaagcttagcgttggcattttcaaaattcaaggtgataacgctttcttcttcctttctgttttagaatagattgctgtctgatttgaaaaagggaaatagatttgatctcaaatgaatctgtgcccagaagccaggctcagggtattcagagatttgtatagtgccctcaaaaaataacaaaattttagctttccttttttcttcttttctccatcaaattcttttttctctagtttacaaatgacatggaaaaggaatttcccctgagttttgtatgcctttttttttttggcttagactatagataggcgtgttgagctcctaagaaaatacaaggaggaactctttgttgtgcagagcactttatgagtagtttgtgtggataatatgtgactgcttccctgacgagcttgtgaggctgtacttatgtctttcctgtaaggcagcttcagtgccttctgtagtgtatataaggaaagattacgccttctgaaaaatctcagagcaaccataagattattttaaaatatgtagtatgactgatggactttttcatcattaaattagtctagcatctaaacttttaccactgaaataatattgaccaaaaagcaatttataaaaggtatttgtgaatagaaaatacaatgtgatcatttgtacttatgtgcaccttaaaagaggaattctgtctagctgtcaaattctggttccttaacatccagtccttgattgtgattgagatctggtaggacgtgctggggcacgctagcagataaaatcccgtatactttaggatagatgttacatttatgtcagtgttggcaaagagcattgtgtagtaataaagaattcaagacttcagcaatgtcaacctgaaactttgtaaatatttcctagattgttatttgatgcagtcacagctctttatcacacaatgttgtctttccctcatcaggcaattttagaactgctgcacacccctcctcagatctcacctgcccctcctgtacattcacctctccagccttgtgcacacctcatttagctttagtttgaaacacattgcagggttcaggtgacctcttcaaaaactacctcctcagaatgaggtaatgaatagttatttattttaaaatatgaaaagtcaggagctctagaatatgaagatgatctaagattttaacttttatgtatacttgttgagcactctccttttgtcctaaagggcattatacatttaagcagtaatactgaaaaatgtagctcagagtaactgaatgttgttgaaagtggtgccagaatctgttttaggggtacgtatcagaatcttaatcttaaatcggttacatgaaattaaatagttaatggtaacacttgactaacagatataattttaattttcggtaggcttttagcaagacagtaagtacatcttcataatgagttagccacagcttcatcacatgcacagattttcctgttgagagactgcccagttaagagggtagaatgatgaaccatttttcaggattctcttctttgtccaaactggcattgtgagtgctagaatatcagcactttcaaactagtgattccaactattaggctattaaaaagcaaaacaaaccaaacaaaccatagccagacatgggaagtttactatgagtataaacagcaaatagcttacaggtcatacattgaaatggtgtaggtaaggcgttagaaaaataccttgacaatttgccaaatgatcttactgtgccttcatgatgcaataaaaaaaaaaaaaatttagcataaatcagtgatttgtgaagagagcagccaccctggtctaactcagctgtgttaatattttttagcgtgcaatttagactgcaaagataaatgcactaaagagtttatagccaaaatcacatttaaaaaatgagagaaaacacaggtaaattttcagtgaacaaaattatttttttaaagtacataatccctagtatagtcagatatatttatcacatagagcaaataggttgaaatcacaattcagtgacatttctagagaaactttttctactcccataggttcttcaaagcatggaacttttatataacagaaatgtgtgacggtcattttaaattgctgtagtttggggctgaagtactgtgtgctgggcagcaatcacatgtattaactagtgagaaaggagaaattaagatataggacagaatttgattttcttgttcccagattactgctgccaacctagacactgagtttccagaggctgaaacgtaaacttgcagctcagcaactgttttgcaaagttagtgggactgtcctgcttatgctgttcaaaaatgctctgagggccaggtggggcctccaggggctcctctctgaggggacatcagactagctaacgacctggcgggcggatgtgaaccggacacactccatggtgtgcttcttgtatcggtccctcgccaccctcaagaaaggcttcagcgggttctctagacgtctccactaaggtgtgttactaacagccatgggttgttgagcacccgaggagtgcaatagcatctctgcatgattgtatattggcccgaagagaatgaagtggccagtgtactcatgttccatgttgctagctctggtaaactgaaaatactggtaagatttttgttttatcagtacactagagagtaagctttgttttgttgtttttagataatgttttcacttccatttggaaagacatttaaattgagtttcagtcctaaattttgccagtcatggtaattagcagtttctatcaggtatttttaaggtagaagaggatagaaacataagttctaaaagcttaaggtaaccgtggtttattttaaaatgtttaggggtggttagtctctacctcaaaaaaagtgagtgaatcttttatttcagcattcacaagttcggctgttgtttttgtaatacattttttttttaaccttttgacccccctttacctaagtgtcaatgtagttttattaattactaagtcagtttcattaaaatgtttatttagcagttttgactaattgcaatgattaatatagccagttgtgcatgaggacacagccagtgagtatatctgggttttttttgtgatgctttttttcttaagacttctgtagatttatgaagtactcattgaaaacaactaaaatacgtttattcgtgttaatatggaaaaaaaaaaa

SEQ ID NO: 24 - protein, 766 aa, Bos taurus
MAALSGGGGGGGGGAEQGQALFNGDMEPEAGAAASSAADPAIPEEVWNIKQMIKLTQEHIEALLDKFGGEHNPPSIYLEAYEEYTSKLDALQQREQQLLESLGNGTDFSVSSSASTDTVTSSSSSSLSVLPSSLSVFQNPTDVSRSNPKSPQKPIVRVFLPNKQRTVVPARCGVTVRDSLKKALMMRGLIPECCAVYRIQDGEKKPIGWDTDISWLTGEELHVEVLENVPLTTHNFVRKTFFTLAFCDFCRKLLFQGFRCQTCGYKFHQRCSTEVPLMCVNYDQLDLLFVSKFFEHHPIPQEEASLAETTLPCGSSPSAPPSDSIGPPILTSPSPSKSIPIPQPFRPADEDHRNQFGQRDRSSSAPNVHINTIEPVNIDDLIRDQGFRSDGGSTTGLSATPPASLPGSLSNVKALQKSPGPQRERKSSSSSEDRNRMKTLGRRDSSDDWEIPDGQITVGQRIGSGSFGTVYKGKWHGDVAVKMLNVTAPTPQQLQAFKNEVGVLRKTRHVNILLFMGYSTKPQLAIVTQWCEGSSLYHHLHIIETKFEMIKLIDIARQTAQGMDYLHAKSIIHRDLKSNNIFLHEDLTVKIGDFGLATVKSRWSGSHQFEQLSGSILWMAPEVIRMQDKNPYSFQSDVYAFGIVLYELMTGQLPYSNINNRDQIIFMVGRGYLSPDLSKVRSNCPKAMKRLMAECLKKKRDERPLFPQILASIELLARSLPKIHRSASEPSLNRAGFQTEDFSLYACASPKTPIQAGGYGEFAAFK

SEQ ID NO: 25 - DNA, 4670 bp, Bos taurus
ggtgtgtcatagtgcagcagattgaatgcagaagatatgaaaattcagatgtcttctgttaaggtgtggaatatcaaacaaatgattaagttgacacaggagcatatagaggccctattggacaaatttggtggggagcataatccaccatcaatatatctggaggcctatgaagaatacaccagcaagctagatgccctccaacaaagagaacaacagttattggaatccctggggaatggaactgatttttctgtttctagctctgcatcaacggacaccgttacatcttcttcctcttctagcctttcagtgctgccttcatctctttcagtttttcaaaatcccacagatgtgtcacggagcaaccccaagtcaccacaaaaacctatcgttagagtcttcctgcccaataaacagaggacagtggtacctgcacggtgtggagtcacagtccgggacagcctgaagaaggcactgatgatgagaggtctaatcccagagtgctgtgctgtttacagaattcaggatggggagaagaaaccaattggctgggacactgatatttcctggcttactggagaggagttgcatgtagaagtgttggagaatgttccacttacaacacacaactttgtacggaaaacttttttcaccttagcattttgtgacttctgtagaaagctgcttttccagggattccgctgtcaaacatgtggttataaatttcaccagcgttgtagtacagaggttccactgatgtgtgttaattatgaccaactagatttgctgtttgtctccaagttctttgaacaccacccaataccacaggaggaggcctccttagcagagactacccttccatgtggctcatccccttctgcacccccctccgattctattgggcccccaattctcaccagtccatctccttcaaaatccattccaattccacagcctttccgaccagcagatgaagatcatcgaaatcagtttggacaacgagaccggtcctcatcagctccaaatgtgcatataaacacaatagaacccgtcaatattgatgacttgattagagaccaagggtttcgtagtgatggaggatcaaccacaggtttatccgccacaccccctgcctcattacctggctcactctctaatgtgaaagcattgcagaaatctccaggacctcagcgagaaagaaagtcctcttcatcctcagaagacaggaatcgaatgaaaacgcttggtagacgggattcaagtgacgattgggagattcctgatggacagatcacagtgggacaaagaattggatcagggtcatttgggacagtctacaagggaaagtggcatggtgatgtggcagtgaaaatgttgaatgtgacagcacccacacctcagcagttacaggccttcaaaaatgaagtaggagtactcaggaaaacgcgacatgtgaatatcctcctcttcatgggttattcaacaaagccacaactggctattgttacccagtggtgtgagggctccagtttatatcatcatctccacatcattgagaccaaattcgagatgatcaaacttatagatattgcacggcagactgcacagggcatggattacttacacgccaagtcaatcatccacagagacctcaagagtaataatatttttcttcatgaagacctcacagtaaaaataggtgattttggtctagccacagtgaaatctcgatggagtgggtcccatcagtttgaacagttgtctggatccattttgtggatggcaccagaagtaatcagaatgcaagataaaaacccatatagctttcagtcagatgtatatgcatttgggattgttctgtatgaattgatgaccggacagttaccttattcaaatatcaacaacagggaccagataatttttatggtgggacgaggatatctgtctccagatctcagtaaggtacggagtaactgtccaaaagccatgaagagattaatggcagagtgcctaaaaaagaaaagagatgaaagaccactctttccccaagtaggaaagactctcctaagcaagagacaaaattcagaagttatcagggaaaaagataagcagattctcgcctctattgagctgctggcccgctcattgccaaaaattcaccgcagtgcatcagaaccctccttgaatcgggctggcttccaaacagaggattttagtctatatgcttgtgcttctccaaaaacacccattcaggcagggggatatgaagcagatttggctcttacatcaaataaaaatagagtagaagttgggatttagagatttcctgacatgcaagaaggaataagcaagaaaaaaaggtttgttttccccaaatcatatctattgtcttttacttctattttttcttaaattttttgtgatttcagagacatgtagagttttattgatacctaaactatgagttcttttttttttttttttttcattattttgatttttttggccaagaggcatatgggatcttagcttgagaaagcaacaattttcttgatgtcattttgggtgagggcacatattgctgtgaacagtgtggtgatagccaccagggaccaaactcacacccgctgcattgaaaggtgaagtcttaaacactggaccagcagagaaattcctactctatgagttctttttgtcatcccctccccgcaccctccacccccaacctaaagtctgatgatgaaatcaacaactattccattagaagcagtagattctggtagcatgatctttagtttgttagtaagattttgtgctttgtggggttgtgtcgttttaaggctaatatttaagtttgtcaaatagaatgctgttcagattgtaaaaatgagtaataaacatctgaagttttttttaagttatttttaacatggtatatacagttgagcttagagtttatcattttctgatattctcttacttagtagatgaattctagccattttttataaagatttctgttaagcaaatcctgttttcacatgggcttcctttaagggattttagattctgctggatatggtgactgctcataagactgttgaaaattacttttaagatgtattagaatacttctgaaaaaaaatagcaaccttaaaaccataagcaaaagtagtaagggtgtttatacatttctagagtccctgtttaggtaatagcctcctatgattgtactttaaatgttttgctctccaaggttttagtaacttggctttttttctaatcagtgccaaactcccccagtttttttaactttaaatatgaggtaataaatcttttacccttccttgatcttttgacttataataccttggtcagttgtttcttaaaaggaatccttaaatggaaagagacaatatcactgtctgcagttctgattagtagttttattcagaatggaaaaacagattattcatttttgaaaattgttcaggggtatgttcattgttaggaccttggactttggagtcagtgcctagctatgcattccaggtctgccattttctggctgtgaaattttggacaagttacttaaccactttaaaccccagctttaagaagtaaattaaccccagtaaattaagaagtaatagcagccacttcgtagagttgttatgaggctcagatgcagtgcaaatgtgtataaagtattcagggagtcacctggtatactataatagacactagaatagttgccaatattatcagcatacaatctgaggattctgtcagccaatcattagcaatctgttgtttgttgggacatgccagtgttctccagttgaaatcagtagcaatctaaaaatggatagattattcctcatttaaatagtgtgttcatataagtgattgcttggatccttatcagaagttgctgttactgaaaaatgataaggctgactaaattgtgatagttgtcagttactaaccaactcccagaaatgaataagaggaacctatctctagttcctagtagaaggtatggacaaaatagtaggtgaaaaataatgtcttgaacccccaaattaagtaagctttaaagagtacaatacctcaaagggtctttgcggtttaaaatttgtatgctgagaatgatgttcattgacatgtgcctatatgtaattttttgatagtttaaaaggtgaaatgaactacagatgggagaggtctgaattttcttgccttcagtcaaatgtgtaatgtggacatattatttgacctgtgaattttatcttttaaaaaagattaattcctgcttcttccttcctaatagttgcattataataatgaaaatgagttgataatttggggggaaagtattctacaaatcaaccttattattttaccattggtttctgagaaattttgttcatttgaaccgtttatagcttgattagaatcatagcatgtaaaacccaactgagggattatctgcagacttaatgtagtattatgtaagttgtcttctttcatttcgaccttttttgcttttgttgttgctagatctgtagtatgtagctagtcacctttcagcgaggtttcagcgaggcttttctgtgtctctaggttatttgagataacttttttaaaattagctcttgtcctcc

SEQ ID NO: 26 - protein, 761 aa, Bos taurus
MKIQMSSVKVWNIKQMIKLTQEHIEALLDKFGGEHNPPSIYLEAYEEYTSKLDALQQREQQLLESLGNGTDFSVSSSASTDTVTSSSSSSLSVLPSSLSVFQNPTDVSRSNPKSPQKPIVRVFLPNKQRTVVPARCGVTVRDSLKKALMMRGLIPECCAVYRIQDGEKKPIGWDTDISWLTGEELHVEVLENVPLTTHNFVRKTFFTLAFCDFCRKLLFQGFRCQTCGYKFHQRCSTEVPLMCVNYDQLDLLFVSKFFEHHPIPQEEASLAETTLPCGSSPSAPPSDSIGPPILTSPSPSKSIPIPQPFRPADEDHRNQFGQRDRSSSAPNVHINTIEPVNIDDLIRDQGFRSDGGSTTGLSATPPASLPGSLSNVKALQKSPGPQRERKSSSSSEDRNRMKTLGRRDSSDDWEIPDGQITVGQRIGSGSFGTVYKGKWHGDVAVKMLNVTAPTPQQLQAFKNEVGVLRKTRHVNILLFMGYSTKPQLAIVTQWCEGSSLYHHLHIIETKFEMIKLIDIARQTAQGMDYLHAKSIIHRDLKSNNIFLHEDLTVKIGDFGLATVKSRWSGSHQFEQLSGSILWMAPEVIRMQDKNPYSFQSDVYAFGIVLYELMTGQLPYSNINNRDQIIFMVGRGYLSPDLSKVRSNCPKAMKRLMAECLKKKRDERPLFPQVGKTLLSKRQNSEVIREKDKQILASIELLARSLPKIHRSASEPSLNRAGFQTEDFSLYACASPKTPIQAGGYEADLALTSNKNRVEVGI

SEQ ID NO: 27 - DNA, 4816 bp, Bos taurus
ctcagctgcgccgggtctcacaagacggttcccgaggtggcccaggcgccgtcccaccgccgacgccgcccgggccgcccgggccgtccctccccgctgccccccgtcctccgcctccgcctccccccgccctcagcctcccttccccctccccgcccagcagcggtcgctcgggcccggctctcggttataagatggcggcgctgagtggcggcggcggcggcggcggcggtggcgcggagcagggccaggctctgttcaacggggacatggagcccgaggccggcgccgcggcctcttcggctgcggaccccgccattcccgaggaggtgtggaatatcaaacaaatgattaagttgacacaggagcatatagaggccctattggacaaatttggtggggagcataatccaccatcaatatatctggaggcctatgaagaatacaccagcaagctagatgccctccaacaaagagaacaacagttattggaatccctggggaatggaactgatttttctgtttctagctctgcatcaacggacaccgttacatcttcttcctcttctagcctttcagtgctgccttcatctctttcagtttttcaaaatcccacagatgtgtcacggagcaaccccaagtcaccacaaaaacctatcgttagagtcttcctgcccaataaacagaggacagtggtacctgcacggtgtggagtcacagtccgggacagcctgaagaaggcactgatgatgagaggtctaatcccagagtgctgtgctgtttacagaattcaggatggggagaagaaaccaattggctgggacactgatatttcctggcttactggagaggagttgcatgtagaagtgttggagaatgttccacttacaacacacaactttgtacggaaaacttttttcaccttagcattttgtgacttctgtagaaagctgcttttccagggattccgctgtcaaacatgtggttataaatttcaccagcgttgtagtacagaggttccactgatgtgtgttaattatgaccaactagagcccccaattctcaccagtccatctccttcaaaatccattccaattccacagcctttccgaccagcagatgaagatcatcgaaatcagtttggacaacgagaccggtcctcatcagctccaaatgtgcatataaacacaatagaacccgtcaatattgatgacttgattagagaccaagggtttcgtagtgatggaggatcaaccacaggtttatccgccacaccccctgcctcattacctggctcactctctaatgtgaaagcattgcagaaatctccaggacctcagcgagaaagaaagtcctcttcatcctcagaagacaggaatcgaatgaaaacgcttggtagacgggattcaagtgacgattgggagattcctgatggacagatcacagtgggacaaagaattggatcagggtcatttgggacagtctacaagggaaagtggcatggtgatgtggcagtgaaaatgttgaatgtgacagcacccacacctcagcagttacaggccttcaaaaatgaagtaggagtactcaggaaaacgcgacatgtgaatatcctcctcttcatgggttattcaacaaagccacaactggctattgttacccagtggtgtgagggctccagtttatatcatcatctccacatcattgagaccaaattcgagatgatcaaacttatagatattgcacggcagactgcacagggcatggattacttacacgccaagtcaatcatccacagagacctcaagagtaataatatttttcttcatgaagacctcacagtaaaaataggtgattttggtctagccacagtgaaatctcgatggagtgggtcccatcagtttgaacagttgtctggatccattttgtggatggcaccagaagtaatcagaatgcaagataaaaacccatatagctttcagtcagatgtatatgcatttgggattgttctgtatgaattgatgaccggacagttaccttattcaaatatcaacaacagggaccagataatttttatggtgggacgaggatatctgtctccagatctcagtaaggtacggagtaactgtccaaaagccatgaagagattaatggcagagtgcctaaaaaagaaaagagatgaaagaccactctttccccaagtaggaaagactctcctaagcaagagacaaaattcagaagttatcagggaaaaagataagcagattctcgcctctattgagctgctggcccgctcattgccaaaaattcaccgcagtgcatcagaaccctccttgaatcgggctggcttccaaacagaggattttagtctatatgcttgtgcttctccaaaaacacccattcaggcagggggatatgaagcagatttggctcttacatcaaataaaaatagagtagaagttgggatttagagatttcctgacatgcaagaaggaataagcaagaaaaaaaggtttgttttccccaaatcatatctattgtcttttacttctattttttcttaaattttttgtgatttcagagacatgtagagttttattgatacctaaactatgagttcttttttttttttttttttcattattttgatttttttggccaagaggcatatgggatcttagcttgagaaagcaacaattttcttgatgtcattttgggtgagggcacatattgctgtgaacagtgtggtgatagccaccagggaccaaactcacacccgctgcattgaaaggtgaagtcttaaacactggaccagcagagaaattcctactctatgagttctttttgtcatcccctccccgcaccctccacccccaacctaaagtctgatgatgaaatcaacaactattccattagaagcagtagattctggtagcatgatctttagtttgttagtaagattttgtgctttgtggggttgtgtcgttttaaggctaatatttaagtttgtcaaatagaatgctgttcagattgtaaaaatgagtaataaacatctgaagttttttttaagttatttttaacatggtatatacagttgagcttagagtttatcattttctgatattctcttacttagtagatgaattctagccattttttataaagatttctgttaagcaaatcctgttttcacatgggcttcctttaagggattttagattctgctggatatggtgactgctcataagactgttgaaaattacttttaagatgtattagaatacttctgaaaaaaaatagcaaccttaaaaccataagcaaaagtagtaagggtgtttatacatttctagagtccctgtttaggtaatagcctcctatgattgtactttaaatgttttgctctccaaggttttagtaacttggctttttttctaatcagtgccaaactcccccagtttttttaactttaaatatgaggtaataaatcttttacccttccttgatcttttgacttataataccttggtcagttgtttcttaaaaggaatccttaaatggaaagagacaatatcactgtctgcagttctgattagtagttttattcagaatggaaaaacagattattcatttttgaaaattgttcaggggtatgttcattgttaggaccttggactttggagtcagtgcctagctatgcattccaggtctgccattttctggctgtgaaattttggacaagttacttaaccactttaaaccccagctttaagaagtaaattaaccccagtaaattaagaagtaatagcagccacttcgtagagttgttatgaggctcagatgcagtgcaaatgtgtataaagtattcagggagtcacctggtatactataatagacactagaatagttgccaatattatcagcatacaatctgaggattctgtcagccaatcattagcaatctgttgtttgttgggacatgccagtgttctccagttgaaatcagtagcaatctaaaaatggatagattattcctcatttaaatagtgtgttcatataagtgattgcttggatccttatcagaagttgctgttactgaaaaatgataaggctgactaaattgtgatagttgtcagttactaaccaactcccagaaatgaataagaggaacctatctctagttcctagtagaaggtatggacaaaatagtaggtgaaaaataatgtcttgaacccccaaattaagtaagctttaaagagtacaatacctcaaagggtctttgcggtttaaaatttgtatgctgagaatgatgttcattgacatgtgcctatatgtaattttttgatagtttaaaaggtgaaatgaactacagatgggagaggtctgaattttcttgccttcagtcaaatgtgtaatgtggacatattatttgacctgtgaattttatcttttaaaaaagattaattcctgcttcttccttcctaatagttgcattataataatgaaaatgagttgataatttggggggaaagtattctacaaatcaaccttattattttaccattggtttctgagaaattttgttcatttgaaccgtttatagcttgattagaatcatagcatgtaaaacccaactgagggattatctgcagacttaatgtagtattatgtaagttgtcttctttcatttcgaccttttttgcttttgttgttgctagatctgtagtatgtagctagtcacctttcagcgaggtttcagcgaggcttttctgtgtctctaggttatttgagataacttttttaaaattagctcttgtcctcc

SEQ ID NO: 28 - protein, 757 aa, Bos taurus
MAALSGGGGGGGGGAEQGQALFNGDMEPEAGAAASSAADPAIPEEVWNIKQMIKLTQEHIEALLDKFGGEHNPPSIYLEAYEEYTSKLDALQQREQQLLESLGNGTDFSVSSSASTDTVTSSSSSSLSVLPSSLSVFQNPTDVSRSNPKSPQKPIVRVFLPNKQRTVVPARCGVTVRDSLKKALMMRGLIPECCAVYRIQDGEKKPIGWDTDISWLTGEELHVEVLENVPLTTHNFVRKTFFTLAFCDFCRKLLFQGFRCQTCGYKFHQRCSTEVPLMCVNYDQLEPPILTSPSPSKSIPIPQPFRPADEDHRNQFGQRDRSSSAPNVHINTIEPVNIDDLIRDQGFRSDGGSTTGLSATPPASLPGSLSNVKALQKSPGPQRERKSSSSSEDRNRMKTLGRRDSSDDWEIPDGQITVGQRIGSGSFGTVYKGKWHGDVAVKMLNVTAPTPQQLQAFKNEVGVLRKTRHVNILLFMGYSTKPQLAIVTQWCEGSSLYHHLHIIETKFEMIKLIDIARQTAQGMDYLHAKSIIHRDLKSNNIFLHEDLTVKIGDFGLATVKSRWSGSHQFEQLSGSILWMAPEVIRMQDKNPYSFQSDVYAFGIVLYELMTGQLPYSNINNRDQIIFMVGRGYLSPDLSKVRSNCPKAMKRLMAECLKKKRDERPLFPQVGKTLLSKRQNSEVIREKDKQILASIELLARSLPKIHRSASEPSLNRAGFQTEDFSLYACASPKTPIQAGGYEADLALTSNKNRVEVGI

SEQ ID NO: 29 - DNA, 2499 bp, Bos taurus
ctcagctgcgccgggtctcacaagacggttcccgaggtggcccaggcgccgtcccaccgccgacgccgcccgggccgcccgggccgtccctccccgctgccccccgtcctccgcctccgcctccccccgccctcagcctcccttccccctccccgcccagcagcggtcgctcgggcccggctctcggttataagatggcggcgctgagtggcggcggcggcggcggcggcggtggcgcggagcagggccaggctctgttcaacggggacatggagcccgaggccggcgccgcggcctcttcggctgcggaccccgccattcccgaggaggtgtggaatatcaaacaaatgattaagttgacacaggagcatatagaggccctattggacaaatttggtggggagcataatccaccatcaatatatctggaggcctatgaagaatacaccagcaagctagatgccctccaacaaagagaacaacagttattggaatccctggggaatggaactgatttttctgtttctagctctgcatcaacggacaccgttacatcttcttcctcttctagcctttcagtgctgccttcatctctttcagtttttcaaaatcccacagatgtgtcacggagcaaccccaagtcaccacaaaaacctatcgttagagtcttcctgcccaataaacagaggacagtggtacctgcacggtgtggagtcacagtccgggacagcctgaagaaggcactgatgatgagaggtctaatcccagagtgctgtgctgtttacagaattcaggatggggagaagaaaccaattggctgggacactgatatttcctggcttactggagaggagttgcatgtagaagtgttggagaatgttccacttacaacacacaactttgtacggaaaacttttttcaccttagcattttgtgacttctgtagaaagctgcttttccagggattccgctgtcaaacatgtggttataaatttcaccagcgttgtagtacagaggttccactgatgtgtgttaattatgaccaactagatttgctgtttgtctccaagttctttgaacaccacccaataccacaggaggaggcctccttagcagagactacccttccatgtggctcatccccttctgcacccccctccgattctattgggcccccaattctcaccagtccatctccttcaaaatccattccaattccacagcctttccgaccagcagatgaagatcatcgaaatcagtttggacaacgagaccggtcctcatcagctccaaatgtgcatataaacacaatagaacccgtcaatattgatgacttgattagagaccaagggtttcgtagtgatggaggatcaaccacaggtttatccgccacaccccctgcctcattacctggctcactctctaatgtgaaagcattgcagaaatctccaggacctcagcgagaaagaaagtcctcttcatcctcagaagacaggaatcgaatgaaaacgcttggtagacgggattcaagtgacgattgggagattcctgatggacagatcacagtgggacaaagaattggatcagggtcatttgggacagtctacaagggaaagtggcatggtgatgtggcagtgaaaatgttgaatgtgacagcacccacacctcagcagttacaggccttcaaaaatgaagtaggagtactcaggaaaacgcgacatgtgaatatcctcctcttcatgggttattcaacaaagccacaactggctattgttacccagtggtgtgagggctccagtttatatcatcatctccacatcattgagaccaaattcgagatgatcaaacttatagatattgcacggcagactgcacagggcatggattacttacacgccaagtcaatcatccacagagacctcaagagtaataatatttttcttcatgaagacctcacagtaaaaataggtgattttggtctagccacagtgaaatctcgatggagtgggtcccatcagtttgaacagttgtctggatccattttgtggatggcaccagaagtaatcagaatgcaagataaaaacccatatagctttcagtcagatgtatatgcatttgggattgttctgtatgaattgatgaccggacagttaccttattcaaatatcaacaacagggaccagataatttttatggtgggacgaggatatctgtctccagatctcagtaaggtacggagtaactgtccaaaagccatgaagagattaatggcagagtgcctaaaaaagaaaagagatgaaagaccactctttccccaagtaggaaagactctcctaagcaagagacaaaattcagaagttatcagggaaaaagataagcaggaaaagtatgtttctttagtacattccaggcatttgggattacagtaaaaacaatattctcgcctctattgagctgctggcccgctcattgccaaaaattcaccgcagtgcatcagaa

SEQ ID NO: 30 - protein, 744 aa, Bos taurus
MAALSGGGGGGGGGAEQGQALFNGDMEPEAGAAASSAADPAIPEEVWNIKQMIKLTQEHIEALLDKFGGEHNPPSIYLEAYEEYTSKLDALQQREQQLLESLGNGTDFSVSSSASTDTVTSSSSSSLSVLPSSLSVFQNPTDVSRSNPKSPQKPIVRVFLPNKQRTVVPARCGVTVRDSLKKALMMRGLIPECCAVYRIQDGEKKPIGWDTDISWLTGEELHVEVLENVPLTTHNFVRKTFFTLAFCDFCRKLLFQGFRCQTCGYKFHQRCSTEVPLMCVNYDQLDLLFVSKFFEHHPIPQEEASLAETTLPCGSSPSAPPSDSIGPPILTSPSPSKSIPIPQPFRPADEDHRNQFGQRDRSSSAPNVHINTIEPVNIDDLIRDQGFRSDGGSTTGLSATPPASLPGSLSNVKALQKSPGPQRERKSSSSSEDRNRMKTLGRRDSSDDWEIPDGQITVGQRIGSGSFGTVYKGKWHGDVAVKMLNVTAPTPQQLQAFKNEVGVLRKTRHVNILLFMGYSTKPQLAIVTQWCEGSSLYHHLHIIETKFEMIKLIDIARQTAQGMDYLHAKSIIHRDLKSNNIFLHEDLTVKIGDFGLATVKSRWSGSHQFEQLSGSILWMAPEVIRMQDKNPYSFQSDVYAFGIVLYELMTGQLPYSNINNRDQIIFMVGRGYLSPDLSKVRSNCPKAMKRLMAECLKKKRDERPLFPQVGKTLLSKRQNSEVIREKDKQEKYVSLVHSRHLGLQ

SEQ ID NO: 31 - DNA, 2404 bp, Bos taurus
ctcagctgcgccgggtctcacaagacggttcccgaggtggcccaggcgccgtcccaccgccgacgccgcccgggccgcccgggccgtccctccccgctgccccccgtcctccgcctccgcctccccccgccctcagcctcccttccccctccccgcccagcagcggtcgctcgggcccggctctcggttataagatggcggcgctgagtggcggcggcggcggcggcggcggtggcgcggagcagggccaggctctgttcaacggggacatggagcccgaggccggcgccgcggcctcttcggctgcggaccccgccattcccgaggaggtgtggaatatcaaacaaatgattaagttgacacaggagcatatagaggccctattggacaaatttggtggggagcataatccaccatcaatatatctggaggcctatgaagaatacaccagcaagctagatgccctccaacaaagagaacaacagttattggaatccctggggaatggaactgatttttctgtttctagctctgcatcaacggacaccgttacatcttcttcctcttctagcctttcagtgctgccttcatctctttcagtttttcaaaatcccacagatgtgtcacggagcaaccccaagtcaccacaaaaacctatcgttagagtcttcctgcccaataaacagaggacagtggtacctgcacggtgtggagtcacagtccgggacagcctgaagaaggcactgatgatgagaggtctaatcccagagtgctgtgctgtttacagaattcaggatggggagaagaaaccaattggctgggacactgatatttcctggcttactggagaggagttgcatgtagaagtgttggagaatgttccacttacaacacacaactttgtacggaaaacttttttcaccttagcattttgtgacttctgtagaaagctgcttttccagggattccgctgtcaaacatgtggttataaatttcaccagcgttgtagtacagaggttccactgatgtgtgttaattatgaccaactagatttgctgtttgtctccaagttctttgaacaccacccaataccacaggaggaggcctccttagcagagactacccttccatgtggctcatccccttctgcacccccctccgattctattgggcccccaattctcaccagtccatctccttcaaaatccattccaattccacagcctttccgaccagcagatgaagatcatcgaaatcagtttggacaacgagaccggtcctcatcagctccaaatgtgcatataaacacaatagaacccgtcaatattgatgacttgattagagaccaagggtttcgtagtgatggaggatcaaccacaggtttatccgccacaccccctgcctcattacctggctcactctctaatgtgaaagcattgcagaaatctccaggacctcagcgagaaagaaagtcctcttcatcctcagaagacaggaatcgaatgaaaacgcttggtagacgggattcaagtgacgattgggagattcctgatggacagatcacagtgggacaaagaattggatcagggtcatttgggacagtctacaagggaaagtggcatggtgatgtggcagtgaaaatgttgaatgtgacagcacccacacctcagcagttacaggccttcaaaaatgaagtaggagtactcaggaaaacgcgacatgtgaatatcctcctcttcatgggttattcaacaaagccacaactggctattgttacccagtggtgtgagggctccagtttatatcatcatctccacatcattgagaccaaattcgagatgatcaaacttatagatattgcacggcagactgcacagggcatggattacttacacgccaagtcaatcatccacagagacctcaagagtaataatatttttcttcatgaagacctcacagtaaaaataggtgattttggtctagccacagtgaaatctcgatggagtgggtcccatcagtttgaacagttgtctggatccattttgtggatggcaccagaagtaatcagaatgcaagataaaaacccatatagctttcagtcagatgtatatgcatttgggattgttctgtatgaattgatgaccggacagttaccttattcaaatatcaacaacagggaccagataatttttatggtgggacgaggatatctgtctccagatctcagtaaggtacggagtaactgtccaaaagccatgaagagattaatggcagagtgcctaaaaaagaaaagagatgaaagaccactctttccccaagatctctcttcccaccatagacacaaaaatttcagatggctacaggtttacatgtaaaaaacagaattataacaaatgatttttat

SEQ ID NO: 32 - protein, 726 aa, Bos taurus
MAALSGGGGGGGGGAEQGQALFNGDMEPEAGAAASSAADPAIPEEVWNIKQMIKLTQEHIEALLDKFGGEHNPPSIYLEAYEEYTSKLDALQQREQQLLESLGNGTDFSVSSSASTDTVTSSSSSSLSVLPSSLSVFQNPTDVSRSNPKSPQKPIVRVFLPNKQRTVVPARCGVTVRDSLKKALMMRGLIPECCAVYRIQDGEKKPIGWDTDISWLTGEELHVEVLENVPLTTHNFVRKTFFTLAFCDFCRKLLFQGFRCQTCGYKFHQRCSTEVPLMCVNYDQLDLLFVSKFFEHHPIPQEEASLAETTLPCGSSPSAPPSDSIGPPILTSPSPSKSIPIPQPFRPADEDHRNQFGQRDRSSSAPNVHINTIEPVNIDDLIRDQGFRSDGGSTTGLSATPPASLPGSLSNVKALQKSPGPQRERKSSSSSEDRNRMKTLGRRDSSDDWEIPDGQITVGQRIGSGSFGTVYKGKWHGDVAVKMLNVTAPTPQQLQAFKNEVGVLRKTRHVNILLFMGYSTKPQLAIVTQWCEGSSLYHHLHIIETKFEMIKLIDIARQTAQGMDYLHAKSIIHRDLKSNNIFLHEDLTVKIGDFGLATVKSRWSGSHQFEQLSGSILWMAPEVIRMQDKNPYSFQSDVYAFGIVLYELMTGQLPYSNINNRDQIIFMVGRGYLSPDLSKVRSNCPKAMKRLMAECLKKKRDERPLFPQDLSSHHRHKNFRWLQVYM

SEQ ID NO: 33 - DNA, 2331 bp, Bos taurus
ctcagctgcgccgggtctcacaagacggttcccgaggtggcccaggcgccgtcccaccgccgacgccgcccgggccgcccgggccgtccctccccgctgccccccgtcctccgcctccgcctccccccgccctcagcctcccttccccctccccgcccagcagcggtcgctcgggcccggctctcggttataagatggcggcgctgagtggcggcggcggcggcggcggcggtggcgcggagcagggccaggctctgttcaacggggacatggagcccgaggccggcgccgcggcctcttcggctgcggaccccgccattcccgaggaggtgtggaatatcaaacaaatgattaagttgacacaggagcatatagaggccctattggacaaatttggtggggagcataatccaccatcaatatatctggaggcctatgaagaatacaccagcaagctagatgccctccaacaaagagaacaacagttattggaatccctggggaatggaactgatttttctgtttctagctctgcatcaacggacaccgttacatcttcttcctcttctagcctttcagtgctgccttcatctctttcagtttttcaaaatcccacagatgtgtcacggagcaaccccaagtcaccacaaaaacctatcgttagagtcttcctgcccaataaacagaggacagtggtacctgcacggtgtggagtcacagtccgggacagcctgaagaaggcactgatgatgagaggtctaatcccagagtgctgtgctgtttacagaattcaggatggggagaagaaaccaattggctgggacactgatatttcctggcttactggagaggagttgcatgtagaagtgttggagaatgttccacttacaacacacaactttgtacggaaaacttttttcaccttagcattttgtgacttctgtagaaagctgcttttccagggattccgctgtcaaacatgtggttataaatttcaccagcgttgtagtacagaggttccactgatgtgtgttaattatgaccaactagatttgctgtttgtctccaagttctttgaacaccacccaataccacaggaggaggcctccttagcagagactacccttccatgtggctcatccccttctgcacccccctccgattctattgggcccccaattctcaccagtccatctccttcaaaatccattccaattccacagcctttccgaccagcagatgaagatcatcgaaatcagtttggacaacgagaccggtcctcatcagctccaaatgtgcatataaacacaatagaacccgtcaatattgatgacttgattagagaccaagggtttcgtagtgatggaggatcaaccacaggtttatccgccacaccccctgcctcattacctggctcactctctaatgtgaaagcattgcagaaatctccaggacctcagcgagaaagaaagtcctcttcatcctcagaagacaggaatcgaatgaaaacgcttggtagacgggattcaagtgacgattgggagattcctgatggacagatcacagtgggacaaagaattggatcagggtcatttgggacagtctacaagggaaagtggcatggtgatgtggcagtgaaaatgttgaatgtgacagcacccacacctcagcagttacaggccttcaaaaatgaagtaggagtactcaggaaaacgcgacatgtgaatatcctcctcttcatgggttattcaacaaagccacaactggctattgttacccagtggtgtgagggctccagtttatatcatcatctccacatcattgagaccaaattcgagatgatcaaacttatagatattgcacggcagactgcacagggcatggattacttacacgccaagtcaatcatccacagagacctcaagagtaataatatttttcttcatgaagacctcacagtaaaaataggtgattttggtctagccacagtgaaatctcgatggagtgggtcccatcagtttgaacagttgtctggatccattttgtggatggcaccagaagtaatcagaatgcaagataaaaacccatatagctttcagtcagatgtatatgcatttgggattgttctgtatgaattgatgaccggacagttaccttattcaaatatcaacaacagggaccaggtgctttgtcctccatgggagtgtaataaatgctgtgcaagggcttacttcccatgagagaagtgagtgaccaacagaaggataatttttatggtgggacgaggatatctgtctccagatctcagtaaggtacggagtaactgtccaa

SEQ ID NO: 34 - protein, 681 aa, Bos taurus
MAALSGGGGGGGGGAEQGQALFNGDMEPEAGAAASSAADPAIPEEVWNIKQMIKLTQEHIEALLDKFGGEHNPPSIYLEAYEEYTSKLDALQQREQQLLESLGNGTDFSVSSSASTDTVTSSSSSSLSVLPSSLSVFQNPTDVSRSNPKSPQKPIVRVFLPNKQRTVVPARCGVTVRDSLKKALMMRGLIPECCAVYRIQDGEKKPIGWDTDISWLTGEELHVEVLENVPLTTHNFVRKTFFTLAFCDFCRKLLFQGFRCQTCGYKFHQRCSTEVPLMCVNYDQLDLLFVSKFFEHHPIPQEEASLAETTLPCGSSPSAPPSDSIGPPILTSPSPSKSIPIPQPFRPADEDHRNQFGQRDRSSSAPNVHINTIEPVNIDDLIRDQGFRSDGGSTTGLSATPPASLPGSLSNVKALQKSPGPQRERKSSSSSEDRNRMKTLGRRDSSDDWEIPDGQITVGQRIGSGSFGTVYKGKWHGDVAVKMLNVTAPTPQQLQAFKNEVGVLRKTRHVNILLFMGYSTKPQLAIVTQWCEGSSLYHHLHIIETKFEMIKLIDIARQTAQGMDYLHAKSIIHRDLKSNNIFLHEDLTVKIGDFGLATVKSRWSGSHQFEQLSGSILWMAPEVIRMQDKNPYSFQSDVYAFGIVLYELMTGQLPYSNINNRDQVLCPPWECNKCCARAYFP

SEQ ID NO: 35 - DNA, 2319 bp, Bos taurus
ctcagctgcgccgggtctcacaagacggttcccgaggtggcccaggcgccgtcccaccgccgacgccgcccgggccgcccgggccgtccctccccgctgccccccgtcctccgcctccgcctccccccgccctcagcctcccttccccctccccgcccagcagcggtcgctcgggcccggctctcggttataagatggcggcgctgagtggcggcggcggcggcggcggcggtggcgcggagcagggccaggctctgttcaacggggacatggagcccgaggccggcgccgcggcctcttcggctgcggaccccgccattcccgaggaggtgtggaatatcaaacaaatgattaagttgacacaggagcatatagaggccctattggacaaatttggtggggagcataatccaccatcaatatatctggaggcctatgaagaatacaccagcaagctagatgccctccaacaaagagaacaacagttattggaatccctggggaatggaactgatttttctgtttctagctctgcatcaacggacaccgttacatcttcttcctcttctagcctttcagtgctgccttcatctctttcagtttttcaaaatcccacagatgtgtcacggagcaaccccaagtcaccacaaaaacctatcgttagagtcttcctgcccaataaacagaggacagtggtacctgcacggtgtggagtcacagtccgggacagcctgaagaaggcactgatgatgagaggtctaatcccagagtgctgtgctgtttacagaattcaggatggggagaagaaaccaattggctgggacactgatatttcctggcttactggagaggagttgcatgtagaagtgttggagaatgttccacttacaacacacaactttgtacggaaaacttttttcaccttagcattttgtgacttctgtagaaagctgcttttccagggattccgctgtcaaacatgtggttataaatttcaccagcgttgtagtacagaggttccactgatgtgtgttaattatgaccaactagatttgctgtttgtctccaagttctttgaacaccacccaataccacaggaggaggcctccttagcagagactacccttccatgtggctcatccccttctgcacccccctccgattctattgggcccccaattctcaccagtccatctccttcaaaatccattccaattccacagcctttccgaccagcagatgaagatcatcgaaatcagtttggacaacgagaccggtcctcatcagctccaaatgtgcatataaacacaatagaacccgtcaatattgatgacttgattagagaccaagggtttcgtagtgatggaggatcaaccacaggtttatccgccacaccccctgcctcattacctggctcactctctaatgtgaaagcattgcagaaatctccaggacctcagcgagaaagaaagtcctcttcatcctcagaagacaggaatcgaatgaaaacgcttggtagacgggattcaagtgacgattgggagattcctgatggacagatcacagtgggacaaagaattggatcagggtcatttgggacagtctacaagggaaagtggcatggtgatgtggcagtgaaaatgttgaatgtgacagcacccacacctcagcagttacaggccttcaaaaatgaagtaggagtactcaggaaaacgcgacatgtgaatatcctcctcttcatgggttattcaacaaagccacaactggctattgttacccagtggtgtgagggctccagtttatatcatcatctccacatcattgagaccaaattcgagatgatcaaacttatagatattgcacggcagactgcacagggcatggattacttacacgccaagtcaatcatccacagagacctcaagagtaataatatttttcttcatgaagacctcacagtaaaaataggtgattttggtctagccacagtgaaatctcgatggagtgggtcccatcagtttgaacagttgtctggatccattttgtggatggcaccagaagtaatcagaatgcaagataaaaacccatatagctttcagtcagatgtatatgcatttgggattgttctgtatgaattgatgaccggacagttaccttattcaaatatcaacaacagggaccaggtgctttgtcctccatgggagtgtaataaatgctgtgcaagggcttacttcccatgagagaagtgagtgaccaacagaaggtctgtgcaaggaaaagagacaaagccacggatcagaagcacatggccataactga

SEQ ID NO: 36 - protein, 681 aa, Bos taurus; identical to SEQ ID NO: 34

SEQ ID NO: 37 - DNA, 2661 bp, Bos taurus
tcagctgcgccgggtctcacaagacggttcccgaggtggcccaggcgccgtcccaccgccgacgccgcccgggccgcccgggccgtccctccccgctgccccccgtcctccgcctccgcctccccccgccctcagcctcccttccccctccccgcccagcagcggtcgctcgggcccggctctcggttataagatggcggcgctgagtggcggcggcggcggcggcggcggtggcgcggagcagggccaggctctgttcaacggggacatggagcccgaggccggcgccgcggcctcttcggctgcggaccccgccattcccgaggaggtgtggaatatcaaacaaatgattaagttgacacaggagcatatagaggccctattggacaaatttggtggggagcataatccaccatcaatatatctggaggcctatgaagaatacaccagcaagctagatgccctccaacaaagagaacaacagttattggaatccctggggaatggaactgatttttctgtttctagctctgcatcaacggacaccgttacatcttcttcctcttctagcctttcagtgctgccttcatctctttcagtttttcaaaatcccacagatgtgtcacggagcaaccccaagtcaccacaaaaacctatcgttagagtcttcctgcccaataaacagaggacagtggtacctgcacggtgtggagtcacagtccgggacagcctgaagaaggcactgatgatgagaggtctaatcccagagtgctgtgctgtttacagaattcaggatggggagaagaaaccaattggctgggacactgatatttcctggcttactggagaggagttgcatgtagaagtgttggagaatgttccacttacaacacacaactttgtacggaaaacttttttcaccttagcattttgtgacttctgtagaaagctgcttttccagggattccgctgtcaaacatgtggttataaatttcaccagcgttgtagtacagaggttccactgatgtgtgttaattatgaccaactagatttgctgtttgtctccaagttctttgaacaccacccaataccacaggaggaggcctccttagcagagactacccttccatgtggctcatccccttctgcacccccctccgattctattgggcccccaattctcaccagtccatctccttcaaaatccattccaattccacagcctttccgaccagcagatgaagatcatcgaaatcagtttggacaacgagaccggtcctcatcagctccaaatgtgcatataaacacaatagaacccgtcaatattgatgacttgattagagaccaagggtttcgtagtgatggaggatcaaccacaggtttatccgccacaccccctgcctcattacctggctcactctctaatgtgaaagcattgcagaaatctccaggacctcagcgagaaagaaagtcctcttcatcctcagaagacaggaatcgaatgaaaacgcttggtagacgggattcaagtgacgattgggagattcctgatggacagatcacagtgggacaaagaattggatcagggtcatttgggacagtctacaagggaaagtggcatggtgatgtggcagtgaaaatgttgaatgtgacagcacccacacctcagcagttacaggccttcaaaaatgaagtaggagtactcaggaaaacgcgacatgtgaatatcctcctcttcatgggttattcaacaaagccacaactggctattgttacccagtggtgtgagggctccagtttatatcatcatctccacatcattgagaccaaattcgagatgatcaaacttatagatattgcacggcagactgcacagggcatggattacttacacgccaagtcaatcatccacagagacctcaagagtaataatatttttcttcatgaagacctcacagtaaaaataggtgattttggtctagccacagtgaaatctcgatggagtgggtcccatcagtttgaacagttgtctggatccattttgtggatggcaccagaagtaatcagaatgcaagataaaaacccatatagctttcagtcagatgtatatgcatttgggattgttctgtatgaattgatgaccggacagttaccttattcaaatatcaacaacagggaccagtctgtgcaaggaaaagagacaaagccacggatcagaagcacatggccataactgaagattttgtgaactctcacaaggaaaaaatttgctctttgaacaataagaaggaactcactaaaatgtaactgagaactgttcaacaggttgaaagctgaaagatgccattggaactgacaaaatgtttcttaaacataaatgatgaaacagtgaaactacataatatctcctctggctgaaacattcaagaagtttaaaatgcttaagttaaaaataaaatcctagtaaacaatggacttactgtgcaacatagagaatatcttacgataacctgtaatggaaaagaatctgaaaaagaatgtatataactgaatcactttgctgtaaactagaatctgacacaacactgtaaatcactacacttttctgttgcatgccaaagattatttaataacgtcattaaaaaattattttaataatta

SEQ ID NO: 38 - protein, 679 aa, Bos taurus
MAALSGGGGGGGGGAEQGQALFNGDMEPEAGAAASSAADPAIPEEVWNIKQMIKLTQEHIEALLDKFGGEHNPPSIYLEAYEEYTSKLDALQQREQQLLESLGNGTDFSVSSSASTDTVTSSSSSSLSVLPSSLSVFQNPTDVSRSNPKSPQKPIVRVFLPNKQRTVVPARCGVTVRDSLKKALMMRGLIPECCAVYRIQDGEKKPIGWDTDISWLTGEELHVEVLENVPLTTHNFVRKTFFTLAFCDFCRKLLFQGFRCQTCGYKFHQRCSTEVPLMCVNYDQLDLLFVSKFFEHHPIPQEEASLAETTLPCGSSPSAPPSDSIGPPILTSPSPSKSIPIPQPFRPADEDHRNQFGQRDRSSSAPNVHINTIEPVNIDDLIRDQGFRSDGGSTTGLSATPPASLPGSLSNVKALQKSPGPQRERKSSSSSEDRNRMKTLGRRDSSDDWEIPDGQITVGQRIGSGSFGTVYKGKWHGDVAVKMLNVTAPTPQQLQAFKNEVGVLRKTRHVNILLFMGYSTKPQLAIVTQWCEGSSLYHHLHIIETKFEMIKLIDIARQTAQGMDYLHAKSIIHRDLKSNNIFLHEDLTVKIGDFGLATVKSRWSGSHQFEQLSGSILWMAPEVIRMQDKNPYSFQSDVYAFGIVLYELMTGQLPYSNINNRDQSVQGKETKPRIRSTWP

SEQ ID NO: 39 - DNA, 7434 bp, Bos taurus
acaccgttacatcttcttcctcttctagcctttcagtgctgccttcatctctttcagtttttcaaaatcccacagatgtgtcacggagcaaccccaagtcaccacaaaaacctatcgttagagtcttcctgcccaataaacagaggacagtggtacctgcacggtgtggagtcacagtccgggacagcctgaagaaggcactgatgatgagaggtctaatcccagagtgctgtgctgtttacagaattcaggatggggagaagaaaccaattggctgggacactgatatttcctggcttactggagaggagttgcatgtagaagtgttggagaatgttccacttacaacacacaactttgtacggaaaacttttttcaccttagcattttgtgacttctgtagaaagctgcttttccagggattccgctgtcaaacatgtggttataaatttcaccagcgttgtagtacagaggttccactgatgtgtgttaattatgaccaactagatttgctgtttgtctccaagttctttgaacaccacccaataccacaggaggaggcctccttagcagagactacccttccatgtggctcatccccttctgcacccccctccgattctattgggcccccaattctcaccagtccatctccttcaaaatccattccaattccacagcctttccgaccagcagatgaagatcatcgaaatcagtttggacaacgagaccggtcctcatcagctccaaatgtgcatataaacacaatagaacccgtcaatattgatgacttgattagagaccaagggtttcgtagtgatggaggatcaaccacaggtttatccgccacaccccctgcctcattacctggctcactctctaatgtgaaagcattgcagaaatctccaggacctcagcgagaaagaaagtcctcttcatcctcagaagacaggaatcgaatgaaaacgcttggtagacgggattcaagtgacgattgggagattcctgatggacagatcacagtgggacaaagaattggatcagggtcatttgggacagtctacaagggaaagtggcatggtgatgtggcagtgaaaatgttgaatgtgacagcacccacacctcagcagttacaggccttcaaaaatgaagtaggagtactcaggaaaacgcgacatgtgaatatcctcctcttcatgggttattcaacaaagccacaactggctattgttacccagtggtgtgagggctccagtttatatcatcatctccacatcattgagaccaaattcgagatgatcaaacttatagatattgcacggcagactgcacagggcatggattacttacacgccaagtcaatcatccacagagacctcaagagtaataatatttttcttcatgaagacctcacagtaaaaataggtgattttggtctagccacagtgaaatctcgatggagtgggtcccatcagtttgaacagttgtctggatccattttgtggatggcaccagaagtaatcagaatgcaagataaaaacccatatagctttcagtcagatgtatatgcatttgggattgttctgtatgaattgatgaccggacagttaccttattcaaatatcaacaacagggaccagataatttttatggtgggacgaggatatctgtctccagatctcagtaaggtacggagtaactgtccaaaagccatgaagagattaatggcagagtgcctaaaaaagaaaagagatgaaagaccactctttccccaagtaggaaagactctcctaagcaagagacaaaattcagaagttatcagggaaaaagataagcagattctcgcctctattgagctgctggcccgctcattgccaaaaattcaccgcagtgcatcagaaccctccttgaatcgggctggcttccaaacagaggattttagtctatatgcttgtgcttctccaaaaacacccattcaggcagggggatatggagaatttgcagccttcaagtagccacaccatcatgacagcatctactcttatttcttaagtcttgtgttcgtacaatttgttaacatcaaaacacagttctgttcctcaactctttttaaagttaaaatttttcagtgcataagctggtgtggaacagaaggaaatttcccatccaacaaaagagggaagaatgttttaggaaccagaattctctgctgccagtgtttcttcttcaacacaaatatcacaagtctgcccactcccaggaagaaagaggagagaccctgagttctgaccttttgatggtcaggcatgatggaaagaaactgctgctacagcttgggagatttgctctgggaagtctgccagtcaactttgcccttctaaccaccagatcaatatgtggctgatcatctgatggggcagttgcaatcaccaagccttgttctctttcctgttctgggattgtgttgtggaacccttttccctagccaccaccagttcatttctgagggatggaacaaaaatgcagcatgcccttcctgtgtggtgcatgttcagtccttgacaaatttttaccaaaatgaagctactttatttaaaaggagggtgagaggtgaggaggtcactttgggtgtggcggaaagggaatgctgcatctttttcctgggctgctggggctctggccttggcttgccagccggaagcgctggcacgcatcgccttcttttcccattgggtccagcaatgaagacgagtgtttggggttttttttttctccaccatgtagcaagttctcaggaaaatacaattgatatcttcctcctaagctcttccaatcagtcaccaagtacttatgtggttactttgtccagggcacaaaatgcctgtatctaattaaaagcctacaaaactgcttgataacagttttgaatgtgagacatttatgtaatttaaatgtaaggtacaagttttaatttctgagtttcttctattatatttttattaaaaaaagaaaataattttcagattgaattggagtaaaataatattacttcccactagaattatatatcctggaaaattgtatttttgttacataagcagcttttaaagaaagatcattacccttttctctacataaatatatggggagtcttagcctaatgacaaatatttataatttttaaattaatggtacttgctggatccatactaacatctttactaatacctcattgtttcttccaacttactcctacactacatcctacatcttcttcctagtcttttatctagaatatgcaacctcaaataaaaatggtggtgtcctcattcattctcctccttccttttttcccaagcctgatcttcaaaaggttggttaatttggcagctgagttcctccccaggcagagaatagaccaattttaggtgtattgggactgagggaggatgtgtaaagattaacatcagtaaagaaccgctgtggagtaattaagaactttgttctttataactggagaatataacctaaccctaacatccctcagcctttactaaagtgtggcgtaaatcacagtagtagcaaagaaagtgactctggatgtgttcctggccagtacctcccttatcatgaatgtagactctctcatcaagatttaggaatataaatcaaatcaaatgtgcccagccaagctatgtagtaagggacttgaacaatattaggcagaacctataaaataaatcagggaattagaaattatttaaagttttcaaattgtaaattgccccggtgtctttcagcctactgccattatttttgctacaatacctacatttcagaggagggcctactgaaaattccatgcaagtggaaaataatcctcaagttattaatgagtttgaaaagcaatgagttcttaagtctttgtgagtagagcaagatcctacaaaattcagaaatagtaaaaatggattcatgctgatttgaagagcatctgtgtgcataatataatgctgcatctcttttaaaagcagtctatttttctttttaaatttgtccccatagatgcttttgaacatgaacatgcttatgttaccttttccgaggttgggaagagccaggagctctcaggcagggccccctccctcagctgggcaggagctgctcaggaggagctagttatagaggaagcttagcgttggcattttcaaaattcaaggtgataacgctttcttcttcctttctgttttagaatagattgctgtctgatttgaaaaagggaaatagatttgatctcaaatgaatctgtgcccagaagccaggctcagggtattcagagatttgtatagtgccctcaaaaaataacaaaattttagctttccttttttcttcttttctccatcaaattcttttttctctagtttacaaatgacatggaaaaggaatttcccctgagttttgtatgcctttttttttttggcttagactatagataggcgtgttgagctcctaagaaaatacaaggaggaactctttgttgtgcagagcactttatgagtagtttgtgtggataatatgtgactgcttccctgacgagcttgtgaggctgtacttatgtctttcctgtaaggcagcttcagtgccttctgtagtgtatataaggaaagattacgccttctgaaaaatctcagagcaaccataagattattttaaaatatgtagtatgactgatggactttttcatcattaaattagtctagcatctaaacttttaccactgaaataatattgaccaaaaagcaatttataaaaggtatttgtgaatagaaaatacaatgtgatcatttgtacttatgtgcaccttaaaagaggaattctgtctagctgtcaaattctggttccttaacatccagtccttgattgtgattgagatctggtaggacgtgctggggcacgctagcagataaaatcccgtatactttaggatagatgttacatttatgtcagtgttggcaaagagcattgtgtagtaataaagaattcaagacttcagcaatgtcaacctgaaactttgtaaatatttcctagattgttatttgatgcagtcacagctctttatcacacaatgttgtctttccctcatcaggcaattttagaactgctgcacacccctcctcagatctcacctgcccctcctgtacattcacctctccagccttgtgcacacctcatttagctttagtttgaaacacattgcagggttcaggtgacctcttcaaaaactacctcctcagaatgaggtaatgaatagttatttattttaaaatatgaaaagtcaggagctctagaatatgaagatgatctaagattttaacttttatgtatacttgttgagcactctccttttgtcctaaagggcattatacatttaagcagtaatactgaaaaatgtagctcagagtaactgaatgttgttgaaagtggtgccagaatctgttttaggggtacgtatcagaatcttaatcttaaatcggttacatgaaattaaatagttaatggtaacacttgactaacagatataattttaattttcggtaggcttttagcaagacagtaagtacatcttcataatgagttagccacagcttcatcacatgcacagattttcctgttgagagactgcccagttaagagggtagaatgatgaaccatttttcaggattctcttctttgtccaaactggcattgtgagtgctagaatatcagcactttcaaactagtgattccaactattaggctattaaaaagcaaaacaaaccaaacaaaccatagccagacatgggaagtttactatgagtataaacagcaaatagcttacaggtcatacattgaaatggtgtaggtaaggcgttagaaaaataccttgacaatttgccaaatgatcttactgtgccttcatgatgcaataaaaaaaaaaaaaatttagcataaatcagtgatttgtgaagagagcagccaccctggtctaactcagctgtgttaatattttttagcgtgcaatttagactgcaaagataaatgcactaaagagtttatagccaaaatcacatttaaaaaatgagagaaaacacaggtaaattttcagtgaacaaaattatttttttaaagtacataatccctagtatagtcagatatatttatcacatagagcaaataggttgaaatcacaattcagtgacatttctagagaaactttttctactcccataggttcttcaaagcatggaacttttatataacagaaatgtgtgacggtcattttaaattgctgtagtttggggctgaagtactgtgtgctgggcagcaatcacatgtattaactagtgagaaaggagaaattaagatataggacagaatttgattttcttgttcccagattactgctgccaacctagacactgagtttccagaggctgaaacgtaaacttgcagctcagcaactgttttgcaaagttagtgggactgtcctgcttatgctgttcaaaaatgctctgagggccaggtggggcctccaggggctcctctctgaggggacatcagactagctaacgacctggcgggcggatgtgaaccggacacactccatggtgtgcttcttgtatcggtccctcgccaccctcaagaaaggcttcagcgggttctctagacgtctccactaaggtgtgttactaacagccatgggttgttgagcacccgaggagtgcaatagcatctctgcatgattgtatattggcccgaagagaatgaagtggccagtgtactcatgttccatgttgctagctctggtaaactgaaaatactggtaagatttttgttttatcagtacactagagagtaagctttgttttgttgtttttagataatgttttcacttccatttggaaagacatttaaattgagtttcagtcctaaattttgccagtcatggtaattagcagtttctatcaggtatttttaaggtagaagaggatagaaacataagttctaaaagcttaaggtaaccgtggtttattttaaaatgtttaggggtggttagtctctacctcaaaaaaagtgagtgaatcttttatttcagcattcacaagttcggctgttgtttttgtaatacattttttttttaaccttttgacccccctttacctaagtgtcaatgtagttttattaattactaagtcagtttcattaaaatgtttatttagcagttttgactaattgcaatgattaatatagccagttgtgcatgaggacacagccagtgagtatatctgggttttttttgtgatgctttttttcttaagacttctgtagatttatgaagtactcattgaaaacaactaaaatacgtttattcgtgttaatatggaaaaaaaaaaa

SEQ ID NO: 40 - protein, 603 aa, Bos taurus
MMRGLIPECCAVYRIQDGEKKPIGWDTDISWLTGEELHVEVLENVPLTTHNFVRKTFFTLAFCDFCRKLLFQGFRCQTCGYKFHQRCSTEVPLMCVNYDQLDLLFVSKFFEHHPIPQEEASLAETTLPCGSSPSAPPSDSIGPPILTSPSPSKSIPIPQPFRPADEDHRNQFGQRDRSSSAPNVHINTIEPVNIDDLIRDQGFRSDGGSTTGLSATPPASLPGSLSNVKALQKSPGPQRERKSSSSSEDRNRMKTLGRRDSSDDWEIPDGQITVGQRIGSGSFGTVYKGKWHGDVAVKMLNVTAPTPQQLQAFKNEVGVLRKTRHVNILLFMGYSTKPQLAIVTQWCEGSSLYHHLHIIETKFEMIKLIDIARQTAQGMDYLHAKSIIHRDLKSNNIFLHEDLTVKIGDFGLATVKSRWSGSHQFEQLSGSILWMAPEVIRMQDKNPYSFQSDVYAFGIVLYELMTGQLPYSNINNRDQIIFMVGRGYLSPDLSKVRSNCPKAMKRLMAECLKKKRDERPLFPQVGKTLLSKRQNSEVIREKDKQILASIELLARSLPKIHRSASEPSLNRAGFQTEDFSLYACASPKTPIQAGGYGEFAAFK

SEQ ID NO: 41 - DNA, 2295 bp, Equus caballus
  misc_feature (79)..(79): n is a, c, g, or t
atgaagacgctgagcggcggcggcggcggcgcggagcagggccaggctctgttcaacggggacatggaacccggaggcnccgcgccggcgcccgcggcctcgtcggccgcggaccctgccattcccgaggaggtatggaatatcaaacaaatgattaaattgacacaggaacatatagaggccctattggacaaatttggtggggagcataatccaccatcaatatatctggaggcctatgaagaatacaccagcaagctagatgccctccaacaaagagaacaacagttattggaatccctggggaatggaactgatttttctgtttctagttctgcatcaacggacaccgttacatcttcttcctcttctagcctttcagtgctaccttcatctctttcagtttttcaaaatcccacagatgtgtcacggagcaaccctaagtcaccacaaaaacctatcgttagagtcttcctgcccaacaaacagaggacagtggtacctgcaaggtgtggcgttacagtccgggacagtctaaagaaagcactgatgatgagaggtctaatcccagagtgctgtgctgtttacagaattcaggatggagagaagaaaccaattggctgggacactgatatttcctggctcactggagaggaattgcatgtagaagtgttggagaatgttccacttacaacacacaactttgtacggaaaacttttttcaccttagcattttgtgacttttgtcgaaagctgcttttccagggtttccgctgtcaaacatgtggttataaatttcaccagcgttgtagtacagaggttccactgatgtgtgttaattatgaccaacttgatttgctgtttgtctccaagttctttgaacaccacccagtatcacaggaggaggcctccttagcagagactgcccttacatctggatcatccccttctgcacccccctccgattccattgggccccaaattctcaccagtccatctccttcaaaatccattccaattccacagcctttccgaccagcagatgaagatcatcgaaatcagtttggacaacgagaccggtcctcatcagctccaaatgtacatataaacacaatagaacctgtcaatattgatgacttgattagagaccaagggtttcgtagtgatggaggatcaaccacaggtttatctgccaccccccctgcctcattacctggctcactcactaatgtgaaggcattacagaaatctccaggacctcaacgggaaaggaaatcatcttcatcctcagaagacaggaatcgaatgaaaactcttggtagacgggattcaagtgacgattgggagattcctgatgggcagatcacagtgggacaaagaattggatctgggtcatttgggacagtctacaagggaaagtggcatggtgatgtggcagtgaaaatgttgaatgtgacagcacccacacctcagcagttacaggccttcaaaaatgaagtaggagtactcaggaaaactcgacatgtgaatatcctactcttcatgggctattcaacaaagccacaactggctattgttacccagtggtgtgagggctccagcttatatcaccatctccacatcattgagaccaaatttgagatgatcaaacttatagatattgctcggcaaactgcacagggcatggattacttacacgccaagtcaatcatccacagagacctcaagagtaataatatttttcttcatgaagacctcacagtaaaaataggtgattttggtctagccacagtgaaatctcgatggagtgggtcccatcagtttgaacagttgtctggatccattttgtggatggcaccagaagtaatcagaatgcaagataaaaacccgtatagctttcaatcagatgtatatgcctttgggattgttctgtatgaattgatgactggacagttaccttattcaaacatcaacaacagggaccagataatttttatggtgggaagaggatatctatctccagatctcagtaaggtacggagtaactgtccaaaagccatgaagagattaatggcagagtgcctaaaaaagaaaagagacgagagaccactcttcccccaaattctcgcctctattgagctgctggcccgctcattgccaaaaattcaccgcagtgcatcagagccctccttgaatcgggctggcttccagacagaggattttagtctatatgcttgtgcttctccgaaaacacccatccaggcagggggatatggtgcgtttcctgtccactga

SEQ ID NO: 42 - protein, 764 aa, Equus caballus
  misc_feature (27)..(27): Xaa can be any naturally occurring amino acid
MKTLSGGGGGAEQGQALFNGDMEPGGXAPAPAASSAADPAIPEEVWNIKQMIKLTQEHIEALLDKFGGEHNPPSIYLEAYEEYTSKLDALQQREQQLLESLGNGTDFSVSSSASTDTVTSSSSSSLSVLPSSLSVFQNPTDVSRSNPKSPQKPIVRVFLPNKQRTVVPARCGVTVRDSLKKALMMRGLIPECCAVYRIQDGEKKPIGWDTDISWLTGEELHVEVLENVPLTTHNFVRKTFFTLAFCDFCRKLLFQGFRCQTCGYKFHQRCSTEVPLMCVNYDQLDLLFVSKFFEHHPVSQEEASLAETALTSGSSPSAPPSDSIGPQILTSPSPSKSIPIPQPFRPADEDHRNQFGQRDRSSSAPNVHINTIEPVNIDDLIRDQGFRSDGGSTTGLSATPPASLPGSLTNVKALQKSPGPQRERKSSSSSEDRNRMKTLGRRDSSDDWEIPDGQITVGQRIGSGSFGTVYKGKWHGDVAVKMLNVTAPTPQQLQAFKNEVGVLRKTRHVNILLFMGYSTKPQLAIVTQWCEGSSLYHHLHIIETKFEMIKLIDIARQTAQGMDYLHAKSIIHRDLKSNNIFLHEDLTVKIGDFGLATVKSRWSGSHQFEQLSGSILWMAPEVIRMQDKNPYSFQSDVYAFGIVLYELMTGQLPYSNINNRDQIIFMVGRGYLSPDLSKVRSNCPKAMKRLMAECLKKKRDERPLFPQILASIELLARSLPKIHRSASEPSLNRAGFQTEDFSLYACASPKTPIQAGGYGAFPVH

SEQ ID NO: 43 - DNA, 2678 bp, Gallus gallus
tccccctccctcgccccagcgcttcgatccaagatggcggcgctgagcagcggcagcagcgccgagggggcctcgctcttcaacggggacatggagcccgagccgccgccgcccgtgctgggcgcctgctacgccgggagcggcggcggcgacccggccatcccggaggaggtgtggaatatcaaacagatgattaaattaacacaagaacatatagaagcgctgttagacaagtttggaggagagcataacccaccatcaatatatttagaggcctatgaggagtacaccagcaaactagatgctctacagcagagagaacagcagttattggaatccatgggaaatggaactgatttctctgtttccagttcagcttcaacggacacagttgcatcatcttcctcctctagcctctctgtagcaccttcatccctttcagtttatcaaaatcctactgatatgtcgcggaataaccctaagtctccacagaagcctattgttagagtcttcctgcccaacaagcaaaggactgtggttccggcaagatgtggggtgacagtccgagacagcctgaagaaagctctgatgatgagaggtcttattccagaatgctgtgctgtttacagaatacaggatggagagaagaagccaattggctgggacactgacatttcctggctaaccggagaggagttacacgtggaggtcttggagaatgtgccactcacaacacacaattttgtacgaaaaacattcttcacgttagcgttctgcgacttctgtcgaaagctgcttttccagggattccgatgccagacatgtggctacaaatttcaccagcgctgtagcacagaagtgccactgatgtgtgttaactacgaccaactcgatttgctgtttgtctccaagttctttgaacatcaccccatatcgcaggaggagaccaccttaggagagaccaccccggcatcgggatcgtacccctcagtgcccccatcagattctgttggaccaccaattctccctagtccttctccttcaaaatccattccaatcccacagcccttccgaccagcagatgaagaccatcggaatcagtttgggcaacgcgaccgatcctcttcagctcccaatgttcacatcaatacaattgagccagtcaatattgatgacttgattagagaccagggtgtacgaggagagggagcccctttgaaccagctgatgcgctgtcttcggaaataccaatcccggactcccagtcccctccttcattctgtccccagtgaaatagtgtttgattttgagcctggcccagtgttcagaggttcaactgcaggtttgtctgcaacacctcctgcatctttgcctgggtcacttaccaatgtgaaagcattacagaaatcaccaggcccccaacgggaaaggaaatcatcctcatcctcagaagacagaaataggatgaaaacccttggtcgacgagattcaagtgatgattgggaaataccagatgggcagatcacagttggacaaaggataggatctggatcatttggaacagtctacaaaggaaagtggcatggtgacgtggcagtgaaaatgttgaatgttacagcacccacacctcaacagttacaggctttcaaaaatgaagtaggagtgctcaggaaaacacggcatgtgaatatcctactttttatgggttattcaacaaaacctcagttggctattgttacacagtggtgtgaggggtccagcttatatcaccatctgcacataattgagaccaagtttgaaatgatcaaactaattgatattgcacgacagactgcacaaggcatggattatttgcatgccaagtcaatcatccacagagacctcaagagtaataatatttttcttcatgaagacctcacagtaaaaataggtgacttcggtctggctacagtgaaatcacgatggagtggatctcatcaatttgaacagttatctggatcaattctatggatggcaccggaagtgatcaggatgcaagacaaaaacccatatagctttcagtcagatgtgtatgcattcgggattgtgctttatgaactgatgactggacagttaccatactcaaacatcaacaacagggaccagataatttttatggtgggacgaggatatctatctccagacctcagtaaagtaagaagtaactgtccaaaagctatgaagagactaatggcagaatgcttgaaaaagaaaagagatgagagacctctttttccacagattcttgcctccattgagcttctggcccggtcgttgccaaaaattcaccgcagtgcatctgagccgtcactaaaccgggctggcttccagaccgaggatttcagtctgtatgcttgtgcttctccaaaaacgcccatccaagcagggggatacggtgggtttccagtacactgaaaagaaatgtgaaagcgtgtgcctgtttgctcatgtgctggtgtgttcctgtgtgtgcaacgcatacgtacgttctcagttcctaccagcgactttttaaggtttactgagggaatgaagactcatttcctaacatggggcattgaacgtcctgagcacaagtcagtgctggtaaggaatgtcttgggaacagctggcaagaagaattagaaggtacttaaagg

SEQ ID NO: 44 - protein, 806 aa, Gallus gallus
MAALSSGSSAEGASLFNGDMEPEPPPPVLGACYAGSGGGDPAIPEEVWNIKQMIKLTQEHIEALLDKFGGEHNPPSIYLEAYEEYTSKLDALQQREQQLLESMGNGTDFSVSSSASTDTVASSSSSSLSVAPSSLSVYQNPTDMSRNNPKSPQKPIVRVFLPNKQRTVVPARCGVTVRDSLKKALMMRGLIPECCAVYRIQDGEKKPIGWDTDISWLTGEELHVEVLENVPLTTHNFVRKTFFTLAFCDFCRKLLFQGFRCQTCGYKFHQRCSTEVPLMCVNYDQLDLLFVSKFFEHHPISQEETTLGETTPASGSYPSVPPSDSVGPPILPSPSPSKSIPIPQPFRPADEDHRNQFGQRDRSSSAPNVHINTIEPVNIDDLIRDQGVRGEGAPLNQLMRCLRKYQSRTPSPLLHSVPSEIVFDFEPGPVFRGSTAGLSATPPASLPGSLTNVKALQKSPGPQRERKSSSSSEDRNRMKTLGRRDSSDDWEIPDGQITVGQRIGSGSFGTVYKGKWHGDVAVKMLNVTAPTPQQLQAFKNEVGVLRKTRHVNILLFMGYSTKPQLAIVTQWCEGSSLYHHLHIIETKFEMIKLIDIARQTAQGMDYLHAKSIIHRDLKSNNIFLHEDLTVKIGDFGLATVKSRWSGSHQFEQLSGSILWMAPEVIRMQDKNPYSFQSDVYAFGIVLYELMTGQLPYSNINNRDQIIFMVGRGYLSPDLSKVRSNCPKAMKRLMAECLKKKRDERPLFPQILASIELLARSLPKIHRSASEPSLNRAGFQTEDFSLYACASPKTPIQAGGYGGFPVH